European Patent Application EP 4 372 103 A1, published May 22, 2024. Title: SUBSTANCE AND METHOD FOR TUMOR ASSESSMENT. Applicant: SINGLERA GENOMICS (JIANGSU) LTD.   SINGLERA GENOMICS (CHINA) LTD. The sequence listing filed with the application follows.

SEQUENCE LISTING (235 sequences)

SEQ ID NO: 1 - DNA, 501 bp, Artificial Sequence
  DMRTA2
agtagggcgccatgaaggccagaccgcggctgtgcgccgccgccgcggagtaggccaggcgcagggggctgaggccgagcggcgcgcccagcgggtaggcgcccgcgtcggcaccgaagtgactggcgttgggctgcagcggcgagaaggccgagcggctgctcagcgagcccagcgccccaggcgccatggcgccggccagcaagggtctgtggtgcggaggtgcggcgggccccgcctgcagcggcgcaggcagcccaggccccccggcggcggcggcggcggcggcggcggcgtcgacgcggctgggccacgcgtcgtctgcagctgctgcagcacccacggcggccttatctgggggcgccgcagggcccaggccggccgccaggcccccacggtggtggttcagcacctgctcgatggcctgcaccacgtcgccgccgcagccctgcaacaccagctccaggacgcctcgccggtggcctgggaacacgcgtgtca

SEQ ID NO: 2 - DNA, 542 bp, Artificial Sequence
  FOXD3
ccctgccccccatctttcgggggcactcaaaccctcttcccctgagctccgtggcagcccccgaacaccctcatcgcccgctgccccctccccgccgccgctaccaaccccgaggagggatgaccctctccggcggcggcagcgccagcgacatgtccggccagacggtgctgacggccgaggacgtggacatcgatgtggtgggcgagggcgacgacgggctggaagagaaggacagcgacgcaggttgcgatagccccgcggggccgccggagctgcgcctggacgaggcggacgaggtgcccccggcggcaccccatcacggacagcctcagccgccccaccagcagcccctgacattgcccaaggaggcggccggagccggggccggaccggggggcgacgtgggcgcgccggaggcggacggctgcaagggcggtgttggcggcgaggagggcggcgcgagcggcggcgggcctggcgcgggcagcggttcggcgggaggcctggccccgagcaagcccaagaacagcctagtgaag

SEQ ID NO: 3 - DNA, 577 bp, Artificial Sequence
  TBX15
atttgttctgcctgatgaaagcaaaagctcgaactcccctcagggcgcgaggtgtgagacccttgggttccatttgcatttctggtttgtcgttggcgggttcctgatttgtttttgttttgttttggtctgttctgttttttggggggtgtctttcaccagggccttcccggttagcccagggtccccacatttctccaggatgtaattagagctaagaacagccgccatccctcagggttccgggtcccgggtttccagggtcccgggtttccaaggccccgcgataaccccgggcgcacgcggcgcgatgcggcgaggcgaggcgaggcggtggggccagcgcggagccccaggcgcgagaacaggaactcgggctggcacaccgaggcctcgcagccaagccgcgcctgacccgttcgccgttccggccccgcggcgcctccaaggccgggccgaggggccgaggggccgagggcgggcagacgcggccacggcctaattctgacttctgaaggtcaccgaaactgcgctgtttttccagagatgggttgaagagaagagatgcaatcccagt

SEQ ID NO: 4 - DNA, 501 bp, Artificial Sequence
  BCAN
atccgctgaacgatgtcctacttcgctcgtccttgctctcgccgctgctgccggagccgaagcagagaaggcagcgggtcccgtgaccgtcccgagagccccgcgctcccgaccagggggcgggggcggccccggggagggcggggcaggggcggggggaagaaagggggttttgtgctgcgccgggagggccggcgccctcttccgaatgtcctgcggccccagcctctcctcacgctcgcgcagtctccgccgcagtctcagctgcagctgcaggactgagccgtgcacccggaggagacccccggaggaggcgacaaacttcgcagtgccgcgacccaaccccagccctgggtaggtgagtgcctccgcagccccgccgcccgccgtggggtcggggacagggagaagggagtgcctgcctggtctgcgccccccgcctgtcagcccttgcctcgaggctctggggcacccaactcgtcgactcctgacaccgcagcg

SEQ ID NO: 5 - DNA, 589 bp, Artificial Sequence
  TRIM58
cttttcaccgggtgtggctcgtctgagctcttgaactgaagccagcggacaccacccgtcggcgcctgctttcctggggcgtgggctcctccccctgtgcagaccgcgaggggagacggtgcgggcggccgggagcgcagccctccgggaggcgggtcatggcctgggcgccgcccggggagcggctgcgcgaggatgcgcggtgcccggtgtgcctggatttcctgcaggagccggtcagcgtggactgcggccacagcttctgcctcaggtgcatctccgagttctgcgagaagtcggacggcgcgcagggcggcgtctacgcctgtccgcagtgccggggccccttccggccctcgggctttcgccccaaccggcagctggcgggcctggtggagagcgtgcggcggctggggttgggcgcggggcccggggcgcggcgatgcgcgcggcacggcgaggacctgagccgcttctgcgaggaggacgaggcggcgctgtgctgggtgtgcgacgccggccccgagcacaggacgcaccgcacggcgccgctgcaggaggccgccggcagctaccaggtgaggcgccc

SEQ ID NO: 6 - DNA, 583 bp, Artificial Sequence
  SIX3
atccaccgtcacactctctccgagcagccagctccccgcttaacggggaaattgaagcagacagcctttgtctaaacacttcttttgcccagaatatcttaattttcctatttgaatgtttaataaggtttggggtgcagcagcttccttttaattgtgacggtgcggccgcttgggcgtgatcccttggctggggctgcagggggcccgtcctccaggggcgcagagggaaggaccagcgtttccaagccgggctctggccgccggcgcgagagcgaggccaaggtctgggggcagttcagggggaccccgaagtcgggacggcccagaaacgctttgcccacagccaccgccctttcctttgtgagtttccccaaagccgtcggtgcgacccggcgccgactctcctcctcttctccctgcgagggcccgcgccgcccgggcccagtcctgggggatagatccctcggggcccaacggctgggccaccgccggtctccggccactgctgcgaggacaggcgctgcctaactaatttctcctctaagggggctgtgcgtgcgtctccttcccaactgatgtc

SEQ ID NO: 7 - DNA, 542 bp, Artificial Sequence
  VAX2
cagaaggtgtcacactctgggatctgttccgcagggaggccacaggtgccaggagacgcgggagagactggctcctgccaagaacatttctttgcattgttcagtgcggttttttatttttatttttgactgtttgtttgcctaagagatgacttcccttgccagaaaaaaaaaagtgttgtaaaaataaaaggaaacgggattacgatgtaaaagacgaatagataaacccggttccgcagatctgcggcgcgcgcgcctggcgacctcggatacattcattgaagttgccgcgcactcgtacccgggttcacctcgcccctcgctcattcctcccgaccaaggcccatggtcagaggtgtcctcgccccgcggccgtcagagggcgcggcctacactcgaatgccggccgagccctccacgcgctcggaacttgggcttcccggtgcagcctccccgcgatcgcaatgcccgctgcctttcccgagcccagtccggaacccgcctctctcggggaccttgacctcgcgcggacctcgtcg

SEQ ID NO: 8 - DNA, 501 bp, Artificial Sequence
  EMX1
cagctccggctctgagcgtctccagtcaggcgaggcggataaatccttcgcaaaaccctcttggaaattgccgccgcttcctgagccatcagtcccagcgggtacgttatcgagtagcacaaacagttggatttttccctcaagaaccgagtctggacgcggagatggagccaagtgtggctgcattttcggacccggaaatccgttgggcactgaaggacttttcgaaccctgtagcgctgttgcttcgcggtccatcgtcgccgctgcagacggatgcgctccccggcggctctacgccctccagtcccggccaggcctctgggctgggagccgagccgtctcgggccctccggcgccgcgttttctagagaaccgggtctcagcgatgctcatttcagccccgtcttaatgcaacaaacgaaaccccacacgaacgaaaaggaacatgtctgcgctctctgcgcagcgcttgggcggcgcggtcccggcgcgcgggga

SEQ ID NO: 9 - DNA, 522 bp, Artificial Sequence
  LBX2
aggaggagagaggtgaggaaaaggctaagtcagagtccgcgaccttgccggctctataccttcagagggctgcagagcgcgcgcgtcaagtccgcggaaagttttactagtcagctcctccagcgcgcacagcggcgacgttggacccggacccgactctggaagctgcggcgcagagggtgctcgggggaccatgcgcggggctaggatgtctgcgatgcttaagagtgtccggggtgttcggggctcgcgtcccgagttcatggtcggccgggctggggcggtccggctgtccgttgcgctaggctccgcaaacgcctgggccccagtgctcggctcccaatccgggcccccagcctcggacccgcccccggctctgggcccgagtcccgtgtgcccctcctcctgcgcccccacctctccaccccgggccgcggtggatctggagctcctagatgtccggggagggtatttctacaggctggggcaggcgcggagagcagaagccgaccaaactaccca

SEQ ID NO: 10 - DNA, 501 bp, Artificial Sequence
  TLX2
caggtgctggagttggagcggcgcttcctgcgccagaagtacctggcctctgcggagagggcggcgctggccaaggccttgcgcatgaccgacgcacaggtcaaaacgtggttccagaaccgacgcaccaagtggcggtgaggcgcggcgcgggcgagggcggactggggttcccgagcagggcctggtgagaagcgacgcggcgggcgccccgctgaccccgcgtctccctcccttaggcgccagacggcggaggagcgcgaggccgagcggcaccgcgcgggccggctgctcctgcatctgcagcaggacgcgttgccacggccgctgcggccgccgctgcccccggaccctctctgcctgcacaactcgtcgctcttcgcgctgcagaacctgcagccctgggccgaggacaacaaagtggcttcagtgtccgggctcgcctcggtggtgtgagcgacgcccgtccgatcggcgtggagcgccgggcccggagcggtg

SEQ ID NO: 11 - DNA, 501 bp, Artificial Sequence
  POU3F3
cggactgtggcccagcccacagaccagggcccgaaattgaggtggggggcgtactctgtttgtcttcccgaaggatgcggcgcgtggaaggagatgcgctgacttgttccaacccataacctttcgctcgggtccccatgtgcgggcagaagaagtcagagcggaacagcctagtgcactggcagggctcattgtctgggaagacaccgaggtctaggcagctgggactgcggagtggaggcaaggccggaggcggccggcggctttgtggaagtttcgcgccgccaggccctgcgcgccgcacggggcggtggagttcttgggcagcccccggcgcttggcccacgcctccgcttcccgcgtgtgggaaactcgagcaccctacaggcaccagggtaaactgcctgtgcctggcccggtgagggtcgctcccccaggccccgtctccgcccgaggactgcaggcctaggcctgcggggagatcctgagaccgcggtgtgc

SEQ ID NO: 12 - DNA, 503 bp, Artificial Sequence
  POU3F3
ggcccgaaattgaggtggggggcgtactctgtttgtcttcccgaaggatgcggcgcgtggaaggagatgcgctgacttgttccaacccataacctttcgctcgggtccccatgtgcgggcagaagaagtcagagcggaacagcctagtgcactggcagggctcattgtctgggaagacaccgaggtctaggcagctgggactgcggagtggaggcaaggccggaggcggccggcggctttgtggaagtttcgcgccgccaggccctgcgcgccgcacggggcggtggagttcttgggcagcccccggcgcttggcccacgcctccgcttcccgcgtgtgggaaactcgagcaccctacaggcaccagggtaaactgcctgtgcctggcccggtgagggtcgctcccccaggccccgtctccgcccgaggactgcaggcctaggcctgcggggagatcctgagaccgcggtgtgcgggcgccggcagcagggcaaggcagggac

SEQ ID NO: 13 - DNA, 504 bp, Artificial Sequence
  TBR1
cttacgcggcggcgggcgtgaaggcgctgccgctgcaggctgcaggctgcactggccgcccgctcggctactacgccgacccgtcgggctggggcgcccgcagtcccccgcagtactgcggcaccaagtcgggctcggtgctgccctgctggcccaacagcgccgcggccgccgcgcgcatggccggcgccaatccctacctgggcgaggaggccgagggcctggccgccgagcgctcgccgctgccgcccggcgccgccgaggacgccaagcccaaggacctgtccgattccagctggatcgagacgccctcctcgatcaagtccatcgactccagcgactcggggatttacgagcaggccaagcggaggcggatctcgccggccgacacgcccgtgtccgagagttcgtccccgctcaagagcgaggtgctggcccagcgggactgcgagaagaactgcgccaaggacattagcggctactatggcttctactcgcacagct

SEQ ID NO: 14 - DNA, 507 bp, Artificial Sequence
  EVX2
tgaggcacgagcagggtgcagagccgccgctggggggcgcgccggccgccgccgccgaggaggccgcagccgctgcggctgccgcggctgccgcggcagaggccgcgctgttgagccccgcggcggccgcgggagcctggtagagaccagggtggcggaagctacacagcagctccggccgagagtaggggtgcgagagggcgcggaaggtgtccagtggccggatggaagtagcgaagggcgacgaagccgcggccgccgcgcctgaggctgcagccgcggccgccgccgccgtgacgcccacgtgcgggtagtagtgcagcggcacgtgcgagtggaaggggtagggcaggcttccggtggcggccgcgtgcgtcatcatgtaggtgtagaagctggggtcggctgggtgcggccaggacatggccaggcgctgccgcttgtccttcatgcgccggttctggaaccacacctgcggggagagacgcgccgcagcctgggttaggg

SEQ ID NO: 15 - DNA, 501 bp, Artificial Sequence
  EVX2 -2
tggaagtagcgaagggcgacgaagccgcggccgccgcgcctgaggctgcagccgcggccgccgccgccgtgacgcccacgtgcgggtagtagtgcagcggcacgtgcgagtggaaggggtagggcaggcttccggtggcggccgcgtgcgtcatcatgtaggtgtagaagctggggtcggctgggtgcggccaggacatggccaggcgctgccgcttgtccttcatgcgccggttctggaaccacacctgcggggagagacgcgccgcagcctgggttagggagcgccccgtgttcccagctcctgtcccaggacctctgccccttccggacctctgaatggcttggtctacttctctccgaccaagcccaaccccgagtaccctgtggtctcccagctgggaaagtgtggacggcagtgtgtggaccgccgtgggcacaccgtcctcaacgaagagggtcctctcccccgcgtccggctgctgctgctcctcaggctttt

SEQ ID NO: 16 - DNA, 581 bp, Artificial Sequence
  HOXD12
ggccagttggccgcgcttccccctatctcctacccgcgcggcgcgctgccctgggccgccacgcccgcctcctgcgcccccgcgcagcctgcgggcgccactgccttcggcggcttctcgcagccctacctggctggctccgggcctctcggcctgcagcccccaacagccaaagacggacccgaagagcaggctaagttctatgcgcccgaagcggccgctgggccagaggagcgcggtcgtacccggccgtccttcgcccccgagtctagcctggctcctgcagtggctgctctcaaagcggccaagtatgactacgctggtgtgggtcgtgccacgccgggctccacgaccctgctccagggggctccctgcgcccctggcttcaaggacgacaccaagggcccgctcaacttgaacatgacagtgcaggcggcgggcgttgcctcttgcctgcgaccttcactgcccgacggtaaacggtgcccatgctccccgggccggtttgggccgggatgggaggtggggttcaagggagagtgtaaggggaggtgaaccgcctgggggcgggcaatagacag

SEQ ID NO: 17 - DNA, 501 bp, Artificial Sequence
  HOXD8
gtcggcagcctcggcggcgggggcgagattggcgggaggggggcgcggggggggcgcggtaagaggtggcggcgggcagagggtgttttttttcttttccctccagagccggggtttgtaaaccgaggccagagtgtccccgtgggccgagcgcacttttttcttgtccgggtgcgctcagtcactggtgcctgagaggaaacagtggaggcagcggggcaggtcgcctggggcgtcggcgattatattgcggccgagccggggcgcgccgggaaaggccgggagggcggcggcgcgcgggggctgggcgaggccccgcgacccgcgagggaggcggcgcgaagccgaggcggcgggcgcaagagccgggcatgagcgcccagtagctgagcgcccgcggctgcctggcctcagaagcgacgcgcgagcgcgggcgggcggcagcagcgacgtagcccggcggtcccggcggcgagagcagccgccccacaggcccccgcg

SEQ ID NO: 18 - DNA, 515 bp, Artificial Sequence
  HOXD4
gggtggggatgggggggtgggggaggactccattttcagagcagggggaaggctgtggaggagcgggggatttccaaaatgcttgagggttccggacctggtggtgggcccagaagaaggagcacatttggggatcccgcaagcctggggtatgtgggtgtgtttgaggaggtgggtgggagtgagcgtgtgcgccggggagagggcgggagggaggaagcaagcgagcttgggagcgcgcggggagggccgcgggcctcggggcgcgccaggaagtgagcggcggaggcgaggggcctaactagtggccgggcgctgacctgcctgtcctgtctgttttgtctcgcagtgaaccccaactacaccggtggggaacccaagcggtcccgaacggcctacacccggcagcaagtcctagaactggaaaaagaatttcattttaacaggtatctgacaaggcgccgtcggattgaaatcgctcacaccctgtgtctgtcggagcgccagatcaagat

SEQ ID NO: 19 - DNA, 512 bp, Artificial Sequence
  HOXD4 - 2
ctggcgctggcacgcttaattcttttttcccacattgcagaatcattcccaccagccactcggagagtggtgggaatctgtcttggtttaatatttctaaaatataagtttcattgtcccccaggttagcccagccaggactcattgcgcagtcctcctcgccttcctggaggcgccgcaggaagcgggaagtcgcggcttggcggttgctgggcctgtgggatctgcgggtcctgcccagacctggagtcgcacagatcacggcgggcagtggctcagcgcctaggcggctccaggcctcgaaggaccaggttggggtgctcagggatcagagaggggaggtcgctctgggtccgggtcgcctgctacgcgccttttctgtctcagaagtggcggtgactcggctgctgagtccgcggaacgagccacggaatggtggtggtggcggggttttctgaggtgactggccagagctgagagtcgcggcttccacctttgggccggagcgggtc

SEQ ID NO: 20 - DNA, 558 bp, Artificial Sequence
  TOPAZ1
tgggattgatttttggcccccgctgcagcaagttgggggctggtgaggagtgtagcggtgactgggggcggagtgcggactcgcatccgctgtaccaggagcccactgccacctcgggattttttttttaacttggaatttccatatgacaaaaaagaaagaggtttctcctcaatctaacggagccattaacatctattaataacgccgacagggtaagtaacggagccgcgctcctcggggtggtcaccgggctgcgtggtcctcggccggcctcctgcatccgctgcccctgtgcgctccgggccggatgcgcaagggcggcgcggggaccaagcctggctgccggccgcctactcctccccttccctaaggtaaggggtcgttttcacactcaccagagctcctgcgggctgagctcgccccctcccccgacttctttgcggggcattttctcttgctggtgtattacgtgtcatttctcacggggcattgccggccgcttttctgcaactgtcctttcggatttggtgatctggtccggcacagaggctctcc

SEQ ID NO: 21 - DNA, 548 bp, Artificial Sequence
  SHOX2
gagagcaggccttgcgggagtctggacccgaagggcgagactccacagggccaaggaaagcggcctctgtcctccgttagtcttgggggagcagacgcaagaggaggcaagggcgccgcgagctccccggatgcactggtcccacaggccgtgcccgagtggagcactgcgaatggggccaagaaattttggcctttctcgccggacctggctgcctccgcgggcctctccgcctaccgcgctcccgccgcggcccgactcccgcgggtctccgcgccgaacccacctggctcctatcgcacgggacattcccgacccacccacgccgcgtcactgagcctctgtaccgatacccggcgcctccgccagcagggcctggacgcaccgcctcctttgacctcgggcttcccccgcgctccgctgcttggggcagactggccccgagagggagccaccatctcccctgctccagggtctccagggtccgaacccgtgttgggatctgggttaggattagggtttggagcttggagcctgcctgttaggac

SEQ ID NO: 22 - DNA, 503 bp, Artificial Sequence
  DRD5
ctccagggatgcgccaagcacccttcggttttcccggggagaattttccccggcccggggactagggtctggcgctggggcgcccctcggacctgcgggatcgcccctacactctggcgcgctgagggcggtgagcgagggcgccaaggcacaggtggggcgggagtcgagcgcggaggctcggggggcgggacgcggggcctgggagcggccagggaccgcggcagcgcctcagtgccagcctggcgcccgcgactgcctgccccagcccctcagtggcggcttgctctcttctctcgctccgaaccagacacagccgctgccgctgccgtccggcgcgctacagactcccgagaacagccctggctgtcagcgagcaccagccgcttcctgtccccatcgcggagactggaggggcgcaccacggccatggagccagaggcgcttcaggaggcaagagaagtccccgcgcgctccgcagcccggcgcagctcatggtgagc

SEQ ID NO: 23 - DNA, 501 bp, Artificial Sequence
  RPL9
gacccacgcccacctaggcctccccgagcctctgttgcatgccgacgggtggctgaacccatcgacggccgaggccttccaggcctacgctgggctgtgcttccaggagctgggggacctggtgaagctctggatcaccatcaacgagcctaaccggctaagtgacatctacaaccgctctggcaacgacacctacggggcggcgcacaacctgctggtggcccacgccctggcctggcgcctctacgaccggcagttcaggccctcacagcgcggggccgtgtcgctgtcgctgcacgcggactgggcggaacccgccaacccctatgctgactcgcactggagggcggccgagcgcttcctgcagttcgagatcgcctggttcgccgagccgctcttcaagaccggggactaccccgcggccatgagggaatacattgcctccaagcaccgacgggggctttccagctcggccctgccgcgcctcaccgaggccgaaag

SEQ ID NO: 24 - DNA, 553 bp, Artificial Sequence
  RPL9 - 2
tggctgaacccatcgacggccgaggccttccaggcctacgctgggctgtgcttccaggagctgggggacctggtgaagctctggatcaccatcaacgagcctaaccggctaagtgacatctacaaccgctctggcaacgacacctacggggcggcgcacaacctgctggtggcccacgccctggcctggcgcctctacgaccggcagttcaggccctcacagcgcggggccgtgtcgctgtcgctgcacgcggactgggcggaacccgccaacccctatgctgactcgcactggagggcggccgagcgcttcctgcagttcgagatcgcctggttcgccgagccgctcttcaagaccggggactaccccgcggccatgagggaatacattgcctccaagcaccgacgggggctttccagctcggccctgccgcgcctcaccgaggccgaaaggaggctgctcaagggcacggtcgacttctgcgcgctcaaccacttcaccactaggttcgtgatgcacgagcagctggccggcagccgctacgactcggaca

SEQ ID NO: 25 - DNA, 610 bp, Artificial Sequence
  HOPX
aaaagagaagtcggagtttagacagggttttaaaagtcagctaaaggctcccacattgcacctgtggttaacaaccacaggccgtgttgcattctttacctggcacttttcgggataatacaggagcatttaaaaaatagataagtcaatgaatgcacttagggggacatcggctgccgctgccgtcagctgaaatgttagctatctaccgtcttataaaacgccaggaaaaacctctaaaccttagagccggggaattttttaaaaaatcggaaccaaatctccgtggcttcgtgcagcgtgagttctgcagctcgggggacgctgcagtgtgatgtggtggagagagcatgcttcaccgctcctgccatcctgacagcgccctccctcccggcctcagcctcctggttcgccaaaccggaggactgaatttatggctagctggtctctggggcgccttccagctctgacattcccgcctagaatagatcttcccgaaggtttcgcagacagaccagaggggaccgagccgggaaggcgagacagggacaggcgagagacgctgctcccaactcgcagagggagaaagcgtgtatcccgggctgccggg

SEQ ID NO: 26 - DNA, 506 bp, Artificial Sequence
  SFRP2
gaacttctgcccttcccgctactggcaccccaagcagggatgcactgggatgcgtggcaggggcgggatctcctgggagcgtctcagcccagcagggagtggggaagcaagagggaaggcttaccttcctcggtggctggcaggaggtggtcgctgctagcgagggggatgcaaaggtcgttgtcctgggggaaacggtcgcactcaagcatgtcgggccaggggaagccgaaggcggacatgaccggggcgcagcggtccttcacctgcacgcagagcgagtggcatggctggatggtctcgtctaggtcatcgaggcagacgggggcgaagagcgagcacaggaacttcttggtgtccgggtggcactgcttcatgaccagcgggatccaagcgccggcctgctccagcacctccttcatggtctcgtggcccagcaggttgggcagccgcatgttctggtattcgatgccgtggcacagctgcaggttggcagggatgggctt

SEQ ID NO: 27 - DNA, 510 bp, Artificial Sequence
  IRX4
attcgagttcttttgcccttttcagtctaagacgtgggctttctgcaaagcctccccctgccagcgagctctcggagcgcggagcctttagaaattgaggggtttactgtcaaaatgaaaatttcacttcaaattaccttggctgatgctcgctcgccaggccgggggctcccgccgcagccttttgacaggcacatgagccgcgagcttccgaacctcgataatatcatctcgagcgcgaaagtcaatacggtgacagcgcgcggccggatacaatccaattacgctcggctgcccgggcgctcctggggctcggggtccggcggccgagggtccccctcagggcccggtccaggccctgtcgccagggttcagggcaggccccaccacgcgggggactttggtggcccaggggtccccacgaggccgcagtccgggtccgcccagccccaggctcctagaggaaagccgagcctagtgagtccctccaaggccgcccgcccgcaagac

SEQ ID NO: 28 - DNA, 501 bp, Artificial Sequence
  TBX18
acttgcgttaagttcggctcaggctactggattgggcaggaccagctaacccaggtcccgaggggcagtgtgtcacagactgcagcccactccaacctcggctcctggagaaggggcgtcgaatctctcttgggcatgggagggaaagacattccgagttggctgggcggagtggcagccttgagagtgacgagtgacagcaaagcctcgtcctagcaaggccttttaccaacagcgcggcatgccctttcgaggagagcgccaggccctcgcactttgcaagtcaagagagcaaagaaagcggggacagggcgcgtaatcgcaatgtccggtcgcgcgtgtgcacgtgtctgtgtttgcatgtgtgcgtgagcatgtgcacctgctcaagtgtaaatgtgtctgttggcagttggggtctaagtacctgagaatgtgtgtcttctgttgctttaggagattaaaatgtcttttcccagtattgagctacattgaggaaac

SEQ ID NO: 29 - DNA, 555 bp, Artificial Sequence
  OLIG3
aagtccttggactcggccgacagccgggccatgttggctgtggagagagcggacaggtgcggcggcggcggcatctggcagatggtgcaggggcagggcagaccagcccagtgctggaagccgctgcccagctgcagcgcgggcggcgtggagggcgccttgagtagcgagtggggaggccggatggtgccgatggcgggaagtgaggcggcggacagcggtgacgaggcgttgccagatgagagcgcgccgcccaagatggggtgcaccgggtgcacggagttggccgcgtgcgcggggtggccggccgagtggcccacggtcccgcagtgaaaggccgagtggtggcccccatagatctcgccaaccagcctcttcatctcctccagggagctggtgagcatgaggatgtagtttctggcgagcaggagtgtggcgatcttggagagcttgcgcaccgacggcccatgcgcgtagggcatgacttcgcgcagcccgtccatggctaggttcaggtcgtgcatccgcttgcgttcgcgtccgttgatcttcagc

SEQ ID NO: 30 - DNA, 501 bp, Artificial Sequence
  ULBP1
tcaggccaggaggtttctggaaggaccggtgctgtctccccgaacatcgtggtctccccgaacatcgcggcctctccgaacatcgccctctctccgagcaacgcgatctccccgaacatcgcggtctccccgaaaatcgcgatctccccgaacattgccatctcaccgaacatcgcgatctcgccgaacatgcccggctgaaggcactcagttcccctccgcggctcctttccgccgggtctgattcctgcggctgctgcttgccccgcaggccaggaggcttctggtagcaccggcgcgatgcccccgaacatcgcgttctaccccaacatcgcgatccctccgaacatcgtgatcccccccgaacatcgccgtccccccgagtaacgcggtctccccgaacatcgcggtccccccgaacatcgcggtacccccgaacatcgccgtctccccgtacattgcgatcccccgaaacattgcgatctccccgaacatcgcgat

SEQ ID NO: 31 - DNA, 516 bp, Artificial Sequence
  HOXA13
ttggccagccgcgcccggactcctcagagctggcgcaaactccgtcctccaaaactcggctctgggaggcctaagtgactccgaagccggcggcagccgcggcagcggccgtggtggtggaagagctcttttccccgacagtgccactgatcgctcttcactggagctggaaacagccttcgcggaaaggaccggagcatgcgttagaagcagagggagcttggtgaagggctcggctggaaggaggaaacgccttctcgcagtgcgcggccagcccgcgggggacaccggcttgctggactgcaggggcccgtgccacccaggaagtgacctgcgggtcactcagccggggcgctgggcgagcgcgggacggcccggagaattccgtgcggctgcgacgggaaaaggacgaggggtctctgtacccgacgctgccactggcccaaaggaattttacccgcgagcgcccaccccaccctagcttgatgcttacgcccgcaacaaaacaggaaacca

SEQ ID NO: 32 - DNA, 516 bp, Artificial Sequence
  TBX20
agacttcgaaggcagccggagaggagagggcccaccgagcactacggcgggtgcgcacgccccggggcgctcggcaggacgacagtctgcacagcccgaaggcggaaacgagcatcaactgcacaaagtcctggggtcctggagcatcccctccgcgtccttcctccctctggggctggggacagccgggatgtcccaggctgaggtggccaccagccgagcgcggctgctaggacgctggcgtggggagcgcggcgcggaactacggacagtgagccctggcgctcgctgccctgcgccttaatttgctggcggcggcgatcccggaggcccgcagccagtcagcgccgtctcacgtcaccgcttcctgattccgccgccgggggcggggccgcgggccgggcgcggagggcgcgcccagggtgcggcgcccgcgtggcctgtcgccccggctgttcggtaccccagcacaggttcagggaaaagggtgccaccactaggctgacgcagcagcca

SEQ ID NO: 33 - DNA, 501 bp, Artificial Sequence
  IKZF1
agcgccggccgccgcatcccgtgcggggccgcggcgcgatgctgcgctggaatgaggaagcgcggcggcgaggggagggcccgggcgcggtgcgcgcgggggtggcggcggcgcgccgagcgggcccggcgcgggcgagcgggctgcagccggcggcggcgccagcaggtacggcccgcacccgccgccgccccggcggcctttgggggctgagccggagcccggcgcgattgcaaagttttcgtgcgcggcccctctggcccggagttgcggctgagacgcgcgccgcgcgagccgggggactcggcgacggggcggggacgggacgacgcaccctctccgtgtcccgctctgcgcccttctgcgcgccccgctccctgtaccggagcagcgatccgggaggcggccgagaggtgcgcgcggggccgagccggctgcggggcaggtcgagcagggaccgccagcgtgcgtcaccccaaagtttgcggggtggcagggcgc

SEQ ID NO: 34 - DNA, 517 bp, Artificial Sequence
  INSIG1
agagctcccggagggcttggccggccaccgccgcgcggcgctgctcggggactgctactttgcaaggcggcggctgcccctgcggggttcgggttgcagggtcaagtgtcacgtcctccgcaatctccaatattcctgtaatgtatttaaatggacgaattcattacgcggggccgtgtgaatggggcgaggccgcgagcgcggcgcgatcagtagcgcccactaacagttcgttctgcacggcggagcgcgagaccgcggacccacggaagccccctcaatggtgtttgcgtcctcgccgccaccggcttggtagggtcctttagggaaggaggaagagttcaggcacccggacagatcctaatggtctttctgatttttctttcccttcggtccgctttccccgcgacctcctccaccctcagtccgcctttcaaacgtcgtccgcggggatggctgcgcgatggagaaattggtctcgtccagagacgcgcgcacagccgtccccgcgcacacg

SEQ ID NO: 35 - DNA, 562 bp, Artificial Sequence
  SOX7
tctcagccacctgattgatttctcctctcactccacccgcacccagtctccgggtccaggcctccagctccctcacttctggctcttctcaccctgaattttctccttatattttttctttcttcctccgattggcagtcccgcttctccgagtggagtcgctcccgccctctcgcgtccccccctggctgcgctgcgacctgcgaactcccccagtttccctcatctgcacaccctggtgtagaccgaccgtgcgcgccgggcccacgtgcagcctggggactgcaggctgggagctcacggccatctctcggccgcgctcaccgcagctcccctgtcacccggccccctgtgaggagctctgttcccgcgctctcatataagcgccggcacacagtaggcgctcaaggcctgcagaatgagtgagcaaatatagctcagacacctactgaatgaaagtcggcaggtttgactagatcctggaatttaaaatttactgagcgccacccatgtgcggggctccacagaggtgatcctggaaggaggcagcgttgtgggggtg

SEQ ID NO: 36 - DNA, 503 bp, Artificial Sequence
  EBF2
ctcagtgataaccgaagagctactctgaaatgccccccttttcctggtggtgcccgccagccggcaggggaaagcccgagggacctcccagctccttcccggatcgcggcggaggtgtgagcgatgtgttgattattcatatttttaccgagcgcatactctgctgcggccggcgccgccacatttcacacgtacactgacgtacccacatgcacaagcgctcactcggccccgcacgcaagcagcgccccgcgcgcccggggccctcctcggataagggaggggtgacaaaagtctcccgctcactgctgcctacccacccccaacccggctgccttttcctccaggcccccacaaacacccttggctttcagatccaactttcttcctcataatatactagtcaccgcgactcccgcctcccggatttgaggatgggggagactttggcggcgggggtcagctgcaaatatggcaccatctagaatttcattccatttagc

SEQ ID NO: 37 - DNA, 701 bp, Artificial Sequence
  MOS
agtattagcatagagaatccagtaatgtgtcgacaacaagcagatagttcccaaaatgccaacctgtttcaacaaagatgaaaacaccaataaacgaaaagtagaaaaacctatgtggacgcatcaacagatgctgaaaaggcatttcctagaagtcggcagccaaacttggtaattcttgcgtgtgataaaggcagccgtctgttctgctcagaaggggtttcctaacaggaggggccgaatgcaggcgtcacatccacgccgccccaggtcgtacacctaggccgtccgggctgtcccagagccgcaggccccgcatcatccgcgtccttagcgcggggcgcggagcccgcagccaggtgcggccgagacccgcgcgccagggaaagcggcgcagcggacgcgggagaaggctggtgggtacaggttgcctccgggccggagcgcccatgcagggcgagctgcgctccgcacaaaattgcggtgggggcgccagaccgccttgctccgcccctgagcggggcgccccggcccaaccccctgagggaggagggtccaggtgccgcagactcttagcccctggcccggcgtccgcccggcaggttctggcactcctcgttggtaagccccgttatttcgtgcgcagtgtttacagaatataaagttcttcaggaaacgatgttataggagaaacgcctgga

SEQ ID NO: 38 - DNA, 505 bp, Artificial Sequence
  MKX
tcccccaacgccggcgaataattttaaagcaaaggaggcgcggccaggtgggctcccaagctccgcgcagacccttgggccagccttggccgctacccgagcgcctctccaccagaccttggagggaagttgggggaagggcgggagagcaccggcgcccagggcgcaggggccagagcgagcctggcgttccgccgcagccggctgagactcggcgacgcgggggctgtacctgtggctgcggggccgacggccggctgcagggcggctggctctcccgcctcgagactaggcgcactcccatccccgccgcatgttctccacgcgggctccagcgcgctcaccaccgccaccgccgtcgtctcggctttatttacccagcccggcgcgcgccgcccgggaacaggaatagcgaggccttctcatgtttcctgactgccggtcccagccggcgaacatcctgcgggcgcggtatccacgttcccgggcgggtggagaggaagcg

SEQ ID NO: 39 - DNA, 549 bp, Artificial Sequence
  KCNA6
atcccagtaagctctagcacccgggcgcgggtaacgggaagcgcagaaccaaatccccagcgcccaggtcacctccccagacccagccttgcagggaccagggctttagggctcacggacccaacggccaggtcagaccgcgaaccgggaggagcgcgggccccaccctaaagagggcgcagccgggagctggggagcgggtgccgcgctccagagattgtgtcgtgggcgccgtcctagtggcggggagcgcacctccgagggggcatgagatcggagaaatcccttacgctggcggcgccgggggaggtccgtgggccggagggagagcaacaggatgcgggagacttcccggaggccggcgggggcgggggctgctgtagtagcgagcggctggtgatcaatatctccgggctgcgctttgagacacaattgcgcaccctgtcgctgtttccggacacgctgctcggagaccctggccggcgagtccgcttcttcgaccccctgaggaacgagtacttcttcgaccgcaaccggcccagcttcgac

SEQ ID NO: 40 - DNA, 506 bp, Artificial Sequence
  SYT10
ccacgttggccccatggcgggagcggagggcgtaggggaaggagaggcgcgcgaggaggctgcggctgccgcgaggtttgcgccaactctcccgccgcgcgagcgagccgaggcgcgctggaactagagacccggcatggagtgctgaggggaggggggagccgtaaaaaagccaaagcaagccctcgactcgcaagcacgcccccctcctctccccagcgcactggtgtttctggcgggtgcctggcggcgacgcgtccaatcgcagcccggcgcgggcgctaggtgacaggcggcggagcgcgcagacccggctccccgcgtcctctgaagaagggactcgcgagggagggagggagggagggcgggcggcccggcgcccctgccgaggccggggatgctcatcgttgcccagagttggcccgaggagccctctccgttttcccaatacttttccctgcatcagtgcagccatccccgccgcctttgtctctccaacttttcca

SEQ ID NO: 41 - DNA, 560 bp, Artificial Sequence
  AGAP2
ggctgcgcggaagcagcggtgacagcagtggctggactcggagttggtgggagggttagcggaggaggagagccggcaggcggtcccggatgcaagtcactgttgtccaaggtcttactcttgcctttccgaggggacaacttccctcgggctccagccccagccccgaccccaccagaggtcgaagctgtagagccccctcccccggcggcggcggcggtggcggcggcagagaccgaagctccagtcccggcgctgctctttgaccccttgaccctgggcttgccctcgctttcgggccatgacaggcggctacccgcgcccttgcccccgccggctttggctccactcgtggtcacggtcttgcaaggcttgggagccggcggaggaggcgccaccttgagcctccggctgccggtgccagggtgcggagaggatgagccagggatgccgccgcccgcccggccttcgggctccgggccgccccagctcgggctgctgagcagggggcgccgggaggaggtgggggcgcccccaggcttggggtcggggctcagtcc

SEQ ID NO: 42 - DNA, 586 bp, Artificial Sequence
  TBX3
gggttcgaatcgaaaatgtcgacatcttgctaatggtctgcaaacttccgccaattatgactgacctcccagactcggccccaggaggctcgtattaggcagggaggccgccgtaattctgggatcaaaagcgggaaggtgcgaactcctctttgtctctgcgtgcccggcgcgcccccctcccggtgggtgataaacccactctggcgccggccatgcgctgggtgattaatttgcgaacaaacaaaagcggcctggtggccactgcattcgggttaaacattggccagcgtgttccgaaggcttgtgctgggcctggcctccaggagaacccacgaggccagcgctccccggaccccggcattaggcgccagctgccggctatctgcggtctttttctctctgcagacccctcgatcctctttccttcggtctcacactcaacaaaagacagactagagacgttgaaagagcctgcccttcaacagagtcccagaaaagggtgacttaaggggaggagaagggagaaagagggcagattccgggtcagaaaagacccagataatttctggcgtctctgaaatat

SEQ ID NO: 43 - DNA, 501 bp, Artificial Sequence
  CCNA1
ataaagttcgattatttcacctggcttgtcagtcacctatgcaggcgtctgagcccccgggtttccaggagccccccgtataaggaccccagggactcctctccccacgcggccgggccgcccgcccggcccccagcccggagagctgccaccgaccccctcaacgtcccaagccccagctctgtcgcccgcgttccttcctcttcctgggccacaatcttggctttcccgggccggcttcacgcagttgcgcaggagcccgcgggggaagacctctcgtggggacctcgagcacgacgtgcgaccctaaatccccacatctcctctgccgcctcgcaggccacatgcaccgggagccgggcggggcaggcgcggcccgcaaggacccccgcgatggagacgcaacactgccgcgactgcacttggggcagccccgccgcgtcccagccgcctcccggcaggaagcgtaggtgtgtgagccgacccggagcgagccgcgcc

SEQ ID NO: 44 - DNA, 528 bp, Artificial Sequence
  ZIC2
agactccctccttgggaacgtcgaactctctctgccttggggagtggggctcgataaagggtacctaggtcgcaccctggcaggggagcactagagggccgcgaggtcccgggtttcgccatcctgagacccccgcgcggatggcccaggaggggcgcggcggccctgagtcaaggtgggcgggggcaggtgcttccctccaccgcgttgtcctatgccggcgcggtccccaccgcccgacctagcccggcgccggccgagcacggcggccgcgcttcgcactccttcctcccaccgggtccgcaggcccggcttcacgattcccgggccctcgggcatgtgagggacttgagtgaatgcagctccctcaactcactcccgcaaaaccacagccaagagggccttaagtcagagaacccggcctaggagcctcccctagagcctcggcgcgggccccttccccttccccacatcggtcggccgagggagcctagagccggtgggagacgggcagcggcctctcctgat

SEQ ID NO: 45 - DNA, 515 bp, Artificial Sequence
  ZIC2 - 2
ggggctcgataaagggtacctaggtcgcaccctggcaggggagcactagagggccgcgaggtcccgggtttcgccatcctgagacccccgcgcggatggcccaggaggggcgcggcggccctgagtcaaggtgggcgggggcaggtgcttccctccaccgcgttgtcctatgccggcgcggtccccaccgcccgacctagcccggcgccggccgagcacggcggccgcgcttcgcactccttcctcccaccgggtccgcaggcccggcttcacgattcccgggccctcgggcatgtgagggacttgagtgaatgcagctccctcaactcactcccgcaaaaccacagccaagagggccttaagtcagagaacccggcctaggagcctcccctagagcctcggcgcgggccccttccccttccccacatcggtcggccgagggagcctagagccggtgggagacgggcagcggcctctcctgatcctttcctgcggtcatacaagttcctagggtg

SEQ ID NO: 46 - DNA, 517 bp, Artificial Sequence
  CLEC14A
gcaaagcctcccaagtcgtctaggcagttagggagctctgcgcatttgccagcacggaggtacctcccggggcagggacacaacacatcgcccgagagtttgtcccagcgagcgccgatttcgtccgcgatgcaagtaactgagatcgggagctgtccccggcagagcgcactcacctcggtcccaggtggactgaagtccagagcggcgctgtgcagctggaagggcgcgcgatagctcaagttagaggcggccccggggcgcggcgcaggacacaagacctcaaactggtacttgcacaggtagccgttggcgcgcaggtggcatcgcatctccttccagcctgcgggctcgaccccaccggtggcctggagtaccgcgcatctccgcgcggtgcaggagcgttggggctcctccacccactgcagcgtgtcgctttcgagaccgccggggtcggaggacagccaggagaaaccccgcaaaggctcgttctccagggtgcagtgggaacgcctgc

SEQ ID NO: 47 - DNA, 507 bp, Artificial Sequence
  CLEC14A - 2
ccaggtggactgaagtccagagcggcgctgtgcagctggaagggcgcgcgatagctcaagttagaggcggccccggggcgcggcgcaggacacaagacctcaaactggtacttgcacaggtagccgttggcgcgcaggtggcatcgcatctccttccagcctgcgggctcgaccccaccggtggcctggagtaccgcgcatctccgcgcggtgcaggagcgttggggctcctccacccactgcagcgtgtcgctttcgagaccgccggggtcggaggacagccaggagaaaccccgcaaaggctcgttctccagggtgcagtgggaacgcctgcgctccagtgcgacccagaacagcaggtctttggagccccctccgggccctgggcctgcccgcaggagcgcgagcacagcgcgcagctcggcgcccgcacgcacggtgctgagcgccccacctcgcaggatgcaggcctcctcggccgcctgccgcttcatggtagcgtggtgc

SEQ ID NO: 48 - DNA, 517 bp, Artificial Sequence
  OTX2
agacttcttgggagtttgcagagcgacccgtcgcccgcgcccggcgctggcagggaccttcggatggttcttactgggccgatccatggcacaggctgggcctcggcgaacccctcggcccccgcccggccccgagccacgacacctcattgtcctggagcctgggaagggggtgcgcgagcgcgcgggcgagccctgcctctccccgccagagaacagctgaggggccgcggtcccagcgggaggattccggtccctggcccggccgcggccttgggcggagcaggggccactagctgccacttctgcccgccccaggtgcgcgcggagggctacgtggggcgggccgcgacccggcaaagtcatgttgaaaaaacactcttcacgttcgctcggcctggtgaccagggtcggggaccacgacaaccgggggttgggaggctgcgtaattacaacccagggtggtttggattttggggggtggtggatatttaaaaacaaaaaggagatctggaag

SEQ ID NO: 49 - DNA, 550 bp, Artificial Sequence
  C14orf39
aaccacagcccgtgcgcctcccgcagtgggagttcgccggccgactcccaccctcacagcctcctgtcctggcttcccctcgcccgaggctgcaacaccgcatcccccccatcccccgccgcgccctcagcctcgggccgcaccaacccaggggataaggcgactccggtcgctctgaggggcagggccagccagccccctcccacccacgcacacgctccccctcagagccgccggcccagagaaaaaccgccacatgcagctcccttccacacgcacctaaacagctcctctggacccgaacgcccacaccctccctccctggggtcccaaactccactcaggacgccacagcggatcctaactacaaacggtccccggagccctgggctggactcgctcagccccgcccccacgcccctggtaccagccctgagagaccccgcggagcacgccgcgggagccgcagatcgcgctgaagagcagcgagatcgcgctctggacgagacctgcgcggctgcaaccgctccttcttcgcgggtggaagcgc

SEQ ID NO: 50 - DNA, 537 bp, Artificial Sequence
  BNC1
gaggaactccggcaaagccaggcggcggcggggctccgggtctgggcggcggctccggaggagcagcgggagaccccgcagcggcctcctccttctccgcccgcggcccccagcctcgccgccgccgcccggctcccagcacggaaccgacggggcgctcccgagacgggcgagccacgcgctcgcaggtcccaaggccaggctgggcgggactgttaagggagctcgaagtcgggggccgggggcttcccgtcccggcgcttcccatgcaaacccctgaaggaagcggcaggcgcagccgcgggctccgcagcccaggcccacttcctgtcactccaggaaaacctcggagcggcggacgcggctcggcccggcttccagcccagagcccaagcgccttagccccgtcccagcgctttctgaaagacgggccacctcgcgcggagccgcgacaaggactccagggtccgcagtgaagctggtcaaatctgccccgcacacggtcaacgctcggtctgtgtcccggaagctttcgga

SEQ ID NO: 51 - DNA, 592 bp, Artificial Sequence
  AHSP
ggatttcgatgaaatggtccctgaagttgtgctccttctgggactccatccttcagctctccaatctcaacagcctgtattctgttgggatggggtaagaccggtgagcgacggtcaaacgtctgtcccacgtggtaaggcgggaaccgctgctgcctgtactgggggcgatactgggggcggcgcagccgattccgggccccagagaactgcctatcagtggtaggggggtcaaatccttcactgctgccgctcccttcttcctcctcctcccagcgtaatcccggggagggccatggcgccttccatagtagccacgtctgtaacggcgccaatcagcgcgtaacgactgccctccacaggaactccaccccggccagtcacactggctgcttctgcacccttctctccttaaaccacatcaaactctacagtttctccatctcctacactgcgcagatatttctgtgggttattcttcttgatggcagtctgatgtataaatagatcttctttggtgtcatttcgatttataaatccatatccatttctgacgttgaaccatttgacagtgccaaggactttggtggcg

SEQ ID NO: 52 - DNA, 701 bp, Artificial Sequence
  ZFHX3
tctattgtatgtacgtgttgcagtcctttcatttgccacaacatatggattccataaatgcagacatgccgaagtgcatctgtctgggtagttaacatgatctaaacatccctcttcgttccgctaactccggctcttcttcgggctcctcggcagcgctccgggccagccggcccgtgccccaggcttgcagcgcccggcagcctcgtccttttgtggtctctgcacgggatccaaggtgccgcgcggaggaggcgggctgctcgcagtgccggggtcagaggcgccgccaccggcggcctctgcgcgcgcggggaggaaagggttaagctgcccgagcccggggaaggggctgctctcatcctggagcgaggtgcagccaccggcagctgtgatttaggggtcaagtccgagatcacctttctcctgcctctggaaatggcagaagatgagatagggagggagaaactagagagtggcagccaggcgcagcacgtgggctccatccatccgacacccccatcgccccggtccactccctgacccccagacaaatcggacagttcccttttctggtagagatgcggggtgcgcttcttctgagcgtccggaatcgctccatccaaggctctgccctaaggttaagccactgtgccctgagcctcaaccaccagatctcaaaagtttgctctcaatgcgcc

SEQ ID NO: 53 - DNA, 531 bp, Artificial Sequence
  LHX1
aggtcggggcgggcttcgttggaagcgggtggcagcgcgggggggcacgcctcgctctctgtaagccactggagagttggggcgagtagggagaaggctgggagtaaatcaaggggaggcggcgagaccgaggacccaattcacggccctgaataacgggggtagctggtaaggggcagctcccgggcttgcgcccagcctcctccctgcacccaggcccgcgagggctccccgcgatccgcgagttccccgcgtggccttcctcagcccgccgaggtcgcgtcttccctccctttcggtcccgccggcccccggccgggccctgacgtcctgcgccctccccgccgctccgcagattaccagagcgagtactacgggcccgggggcaactacgacttcttcccgcaaggccccccgtcctcgcaggcccagacaccagtggacctacccttcgtgccgtcatctgggccgtccgggacgcccctgggtggcctggagcacccgctgccgggccaccacccgtcgagcgag

SEQ ID NO: 54 - DNA, 554 bp, Artificial Sequence
  TIMP2
tcactggctctacagactgccacgggtaaacagcttagaccagatgactcaggctgaaagcatatgaacccttcctgcagggaggccgcccggatgcaacagtggtttcacccctgagccgggcagccttggcagaccttgcttcacgtgggctgaaatggcagtgtctctcctctttgtggccaggttttgcctcctctttgactcggaagcatctcctatcctgcaaggacagtttgagcagggcccccgggccctccttccaagaggcttctgcagctgtggacccccaagagtttatgccgctgagctctgctgtctctccccacctgctccccacctgtctgcccccacacctgcgactctggctctcctggatcctcctgtagactggttcctataagcacaaggaggaacatgcgagatgctgggattggatgctctgggcctggggctggtgtttcctcatgcccgggctatttccttttggccctgggcatgcagtcatgtgcttcctttcatgggcgggttggggaccagggccagcgagcaga

SEQ ID NO: 55 - DNA, 594 bp, Artificial Sequence
  ZNF750
ggtgcccgtctgtgtgtgctcctcccagcagccatcgctcaaccttgctctcaggaagcccccaggcgagtgttggcaggaatcctgccaggcgggaggtcgctcctccagagcgtggtccctgaagccgccagcctccctggcctcgccccttgctggtggtgtgtgtggtgtggccgtgggtgcactttgctgggtcttcctgggacactgaagtctcctgtgtctccagccctgagaactcggagcccgggtgcttttgggaaggacggggcaccagctggtgacacatgggaagggaggtgtggttgtcaccttgcccaggtaacctgctctgcctggtcggtgcgcctaaggggggcagggtgtttggggaggacatgagaggcctcctggaagcacttcatcctgttgaagttcacattttgaccttttcagcagcccttgctctgggcctgtgcccggccctgggactcggcctggagagcctattgacaccgtgccatgggtgcgggcagggcgccctccctggagggcggcacgtggtgccagttggtgaccatgagctgcctcactcctgaggaagagtgttcg

SEQ ID NO: 56 - DNA, 506 bp, Artificial Sequence
  SIM2
ccgctgcggggatttctcccccagccttttctttttaacagagggcaaaggggcgacggcgagagcacagatggcggctgcggagccggggaggcggcggggagacgcgcgggactcgtggggagggctggcagggtgcaggggttccgcgtgacctgcccggctcccaggcatcgggctgggcgctgcagtttaccgatttgctttcgtccctcgtccaggtttaggagacgcgtggggacagccgagccgcgccgggcccctggacggcgtcgccaaggagctgggatcgcacttgctgcaggtagagcggcctcgccgggggaggagcgcagccgccgcaggctcccttcccaccccgccaccccagcctccaggcgtcccttccccaggagcgccaggcagatccagaggctgccgggggctggggatggggtggtccccactgcggagggatggacgcttagcatgtcggatgcggcctgcggccaaccctaccctaaccc

SEQ ID NO: 57 - DNA, 523 bp, Artificial Sequence
  SIX3 - 2
taatttatggaatccaccgtcacactctctccgagcagccagctccccgcttaacggggaaattgaagcagacagcctttgtctaaacacttcttttgcccagaatatcttaattttcctatttgaatgtttaataaggtttggggtgcagcagcttccttttaattgtgacggtgcggccgcttgggcgtgatcccttggctggggctgcagggggcccgtcctccaggggcgcagagggaaggaccagcgtttccaagccgggctctggccgccggcgcgagagcgaggccaaggtctgggggcagttcagggggaccccgaagtcgggacggcccagaaacgctttgcccacagccaccgccctttcctttgtgagtttccccaaagccgtcggtgcgacccggcgccgactctcctcctcttctccctgcgagggcccgcgccgcccgggcccagtcctgggggatagatccctcggggcccaacggctgggccaccgccggtctccggccactgctgc

SEQ ID NO: 58 - DNA, 518 bp, Artificial Sequence
  TLX2 - 2
aagccgcgcacgtccttctcccgctcacaggtgctggagttggagcggcgcttcctgcgccagaagtacctggcctctgcggagagggcggcgctggccaaggccttgcgcatgaccgacgcacaggtcaaaacgtggttccagaaccgacgcaccaagtggcggtgaggcgcggcgcgggcgagggcggactggggttcccgagcagggcctggtgagaagcgacgcggcgggcgccccgctgaccccgcgtctccctcccttaggcgccagacggcggaggagcgcgaggccgagcggcaccgcgcgggccggctgctcctgcatctgcagcaggacgcgttgccacggccgctgcggccgccgctgcccccggaccctctctgcctgcacaactcgtcgctcttcgcgctgcagaacctgcagccctgggccgaggacaacaaagtggcttcagtgtccgggctcgcctcggtggtgtgagcgacgcccgtccgatcggcgtggagcgccgggcc

SEQ ID NO: 59 - DNA, 526 bp, Artificial Sequence
  CILP2
ttcaagatctaagtgagaggccggtcagacagaggcaagagctcagcgcaccgggatggaccaggtcaggccctgggcggcagaactggggtcgcggggaacccagtctgccctgcacctgtttcaggccgctggctcgggtcgtgggcgcgctcggctagccggtgcccaccgggggagggggctgagacagcaagtaaggcctttgcacgcatgcatgggggcctacaggccgccgccctggtcccagcgcgtgcggtgcccgcagaggccagcgagtggacgtcctggttcaacgtggaccaccccggaggcgacggcgacttcgagagcctggctgccatccgcttctactacgggccagcgcgcgtgtgcccgcgaccgctggcgctggaagcgcgcaccacggactgggccctgccgtccgccgtcggcgagcgcgtgcacttgaaccccacgcgcggcttctggtgcctcaaccgcgagcaaccgcgtggccgccgctgctccaactaccacgtgcgct

SEQ ID NO: 60 - DNA, 200 bp, Artificial Sequence
  ARHGEF16 (-60,185), PRDM16 (+325,030)
ttccgcagcgccgcggatcagaggagggaggcctggcgccctcggagctgcggtggggggcatcccaggagatctggctcggtgtgtagagaagggagtccgggcggcgtcctgggagtgtctgtggcctgcagagaggggatggggttggggtgtggatcccgggaggctcggaggcgctcggaggctctcggaggggg

SEQ ID NO: 61 - DNA, 311 bp, Artificial Sequence
  NFIA (-27,057)
aagatgctttctactaatggagaactttaccccgggtcttgcaacccactaaacttggcgtcccatgccacactgggcgtcccaggcctgcctgccctcgacggggcggtctctctgccggcccctggtaaaacagttactgcacctggggcttcgcagagtgcaaggaggaaagaagtggggcattactttccaacaagcaatgacctcagcctgccagcgcctaccttgttctggaaacacctaatctctgcttcctctataaagtttaactgcagcttgcctccaatcccaaattgcaaacactagca

SEQ ID NO: 62 - DNA, 200 bp, Artificial Sequence
  ST6GALNAC5 (+70)
ttaggacccagcaggcggcggcaggcggcagttgtgtagatcgctgagagactacgagggtccggttcagttttaattctgtctctaatctctgcaacagccgcgcttcccgggtcccgcggctcccgcgcgcgatctgccgcggccggctgctgggcaaaaatcagagccgcctccgccccattacccatcatggaaac

SEQ ID NO: 63 - DNA, 200 bp, Artificial Sequence
  PRRX1 (-2,486)
ggaagggaaaaacggcccacatcgaactggatgccggatggaaacctctctgcgctattagactgcgtccagtacagcagatggcacgagcacgtgcggcgctcagcttaggctctcggaggcagctgagttggaaatcccgacggaaagcacccacaagctcccactctgcgctggcccacccgcgtgcacgcccaccc

SEQ ID NO: 64 - DNA, 365 bp, Artificial Sequence
  LHX4 (+3,243), ACBD6 (+269,425)
gcccccggtgcgggcctcgtcgctccgacagccctacagctgtccctacggcccgcaccgacagctcgtccccgccacctccctccgggctgtagggacgtcgagatccgaatcctcacagcgcctgacccggggccgtgttgggtacgggtacggcgagagccttccgagccgcctccaaaactctccccgcggacctcagcagtccctccacgcgtcggggccctgctggccggccatgccctctgaggagacgcggaaaagagcgaggcatataggaaggtggggcgttttatccgcctcggttttgacccatctgccatgtagtctccccaggcaccgagggaaaggacgacggaagcccg

SEQ ID NO: 65 - DNA, 225 bp, Artificial Sequence
  FMN2 (-93,837), CHRM3 (+368,970)
ggggagcggaacagggaacgggctggtggcggccccaagcgggagggacggaccgacacgcggccccctggcggccttgcgactcgccgacctgcggaacctcgtcgccgccctcacagccccgcggccaccgccgacccgggccggtccccggggcgtcgcgggtgttaaagggcgagtctacgcggatgtcacggtcgccgcgggcaaggaccgcgaggttgc

SEQ ID NO: 66 - DNA, 511 bp, Artificial Sequence
  FAM150B (-180,056), TMEM18 (+209,087)
gaaaccagggcggaggagccgcgaggggcaggacgaggctgcatgggccagcgagggggtcgacaccgagccagagtgagcgcggggcctggggcgcagagcccgcccagggagccgggagacgccgcgcaagctccccggacaaacgcaatgaccgaggacgcgcgggcgaggccgtccagggagccctggtccctcagctgcaccggactgagccgcgaccgctcagcacgcgctgcttataaatcaggggtgcgcttcccaagccccgggtgaggtcccctacgtcggcacagccttaggagctgcaaagcagcgcgcgcctccggggctcctgcgcgccccttgaaccccgcctcccgcatcctcctgcaacagcctggagctccctgtgcaggacgcagcggggggcggggggcggtcttaggaggctgcggggcgcactcccacctcctgcctccccgagacccccagcgccttctccagggtttagagcggaggtgaaggggcc

SEQ ID NO: 67 - DNA, 365 bp, Artificial Sequence
  FAM150B (-181,455), TMEM18 (+207,688)
gtgtgcacattggggagcctccgcatgggtgagttcaatgctctgttcttcgtgctgaaggtggaactcatatgcaatggcgtttatttttcccctgacgactataaattttccctgataatctggggccagagtccactggtgcagcaggtgggatgcgggcggcggatggagtccctgagctggggaggactgtgcagctccctcggtgacgctgagcccgtctgggcattcatgcgatacgcagcgctctttactgcgggtcccatctacaataatgtttatcccgcaggtgtttaattctcatagcacagctaggctagcagagtttttaaggtaaattaaccagaatagacatgatcatg

SEQ ID NO: 68 - DNA, 276 bp, Artificial Sequence
  SIX3 (-12,826), CAMKMT (+566,973)
aacgcggccgaaggtttcggagccaggcttcccgggcgtcaggggctagggacgggtccccggagctggggaagatgaggggccgagaggccgtggaggcggaggacgcgggcaagccacggcccggctgggagcttcgggaagcgccgcgcccgggacgcggtctccgggcggggcgaagcgcagggaaggcggcgagggggtccccacacccgcacggggcaccgggtttgtccatgtgggtgacactgccttcaaggcccaggcccgatgggg

SEQ ID NO: 69 - DNA, 200 bp, Artificial Sequence
  OTX1 (+8,100), WDPCP (+529,896)
cacactgtgaagcggggttcggagaacgacccctcccgcgttccgcgcccagcggggtcgcagggctgcgagcccggctgtagcaaagctttctcggccgcgtcctccctccggattcggtaggccaggctcgggcgcgcccttcccacaccaacaaaccatctttcccgactcagcagaggcccacaggggcgcagccg

SEQ ID NO: 70 - DNA, 200 bp, Artificial Sequence
  OTX1 (+8,317), WDPCP (+529,679)
gcccagcggcgccgccctggtacgccaggcctgaaggcagggccggcccgcgccacgcagggtctcccttaggcggcgccttagggtgaaatgcggggccaagcctgacctgccggggtgccccgtggcatctctggtgcggaccccgcacgtgccggggagaactggcaggcggccagggcgaggaggcttccagcttg

SEQ ID NO: 71 - DNA, 225 bp, Artificial Sequence
  CYP26B1 (+3,846), DYSF (+677,489)
acgaggtggtgctcgcccatgaggatcttgcgcacgttctccgcgccggtcacgcgtatcagcggccgccccaacaaatgcgtcttgaacacgttgccatacttctccctccgcgacgactggaagccagaaccctgcgggagccacacccgggtctctctcagggtgcacttctgcagagggcccgcgagggaggggcggcggaccccaacccggggtacagtc

SEQ ID NO: 72 - DNA, 415 bp, Artificial Sequence
  HOXD1 (-10,037), HOXD4 (+27,320)
tttctctgtgtgtgtctagggttgggggcaggagaggttagttctattaagagttcatcaatcacccggtgtgcacttttcgctcgacagcggttcctcctacttcagagcaagtctgggccagctgggatccgaccagaaatcgcaagcggaggagacgcagtagcgcaggctgagcgctaactgaaggcgcgacctgagcccggcgcctgctggggagctgcgcagccaggacagcggtcggcagcacagggcctgggcgcagggcccgccgtcaccacctcacgtcggaagccagcactgctgcccgccagccctgccgcctgccctcggacttcccagggcgcccagggtcctcccaacgcgcctgcacccacacccgcccctgagccacagtgaccttgcattccccgcc

SEQ ID NO: 73 - DNA, 230 bp, Artificial Sequence
  UBE2F (-10,627), RAMP1 (+96,783)
gtccaaggaccgagctgggagtgggggcggagccaagaaggggcgcccctgcgcccacaagccgcagcgcccaggaatcccctgggcgcctccgcgtcccccgcgggctgtcccggcaggcaggcagcccaccccagggctcccctcgtggaaggacacccctgctgaccctggccctggttctggcggtgtctccactcagccctcggagggacgcccacctcccgcgg

SEQ ID NO: 74 - DNA, 200 bp, Artificial Sequence
  AMT (+554)
tcacctgcagcatatgagacacgtcaaagagcgagcagtgctggcgtgtgtgcaggtgcgagtcagtgtgactgtcccggtactgcactggcagactccaacccgcaaacgccaccattttcccgccgtgggccaggtggaagtcatagagcggtgtcctgcggagcacctcctgtgggcggctgggcttagtgccacca

SEQ ID NO: 75 - DNA, 200 bp, Artificial Sequence
  PLSCR5 (-785,959), ZIC4 (+12,109)
tccgcactgacttgcgatgtcgaccggtctgcccagaccacccccacctggctgtcgggcctctcggtcctaagacgaggggttggcgcggtagggtccgcacaggccaaatgggatccgaggtgtctaccgcaaccacgcccttgagcgctgcggcttcgggaagaaaacagctgctgctgtcaggccaggcctggctc

SEQ ID NO: 76 - DNA, 351 bp, Artificial Sequence
  PEX5L (-371)
gagggcggccccgggcggtgcgcgctccccgagcgcgtcctcggggctgcgcgcgcgcggcggcaaggcgaggtgccggcaggcggtggtcgcgctggtgtacaacgcccgcagcagcgcggcgttcaggtgcggcgtcggcgggcagggcgattctagcggagaggatggccggccggaagaaaggcgggaagacatgcatcgtctctccgggggccatccaccgcggctgagcctgttatcctacagacattataggctgagtgcaggggttgccgaagagtttacttcggttctgattcagctctcgaaagttacgtccgtatcacccgttaaataaagactccccgc

SEQ ID NO: 77 - DNA, 200 bp, Artificial Sequence
  ETV5 (-146,916), DGKG (+106,209)
aaactaatgtttcttcctccttctgtgatcttccttctttctgttttgagcagcttctatcacctgtgtcctctgcggatgaactgcataaagctctccgccaaagcctacttctccctcatggtggagagggagccgtgtgagtagtccggtaccgcagccatccaccctctgcagatcagcttttccttccttggctc

SEQ ID NO: 78 - DNA, 207 bp, Artificial Sequence
  FGF12 (+617)
gggaggcagtgctaaaatttgaggaggctgcagtatcgaaaacccggcgctcacaaggttagtcaaagtctgggcagtggcgacaaaatgtgtgaaaatccagatgtaaacttccccaacctctggcggccggggggcggggcggggcggtcccaggccctcttgcgaagtagacgtttgcaccccaaacttgcaccccaaggcgat

SEQ ID NO: 79 - DNA, 200 bp, Artificial Sequence
  FGFRL1 (+12,106), RNF212 (+91,441)
tgtttgctgggccagtgctcagggctttggtgcatgtgggcagctgaggcctgggtcaggggcactgcacctcggcccctctgctcatcttgggcaggtgacccaggtggagctcaggcccgaggtctgtgctgggccgtgggtccccttttgaccgcccccccggctccggaccccaagcccctcctcgctgactgttc

SEQ ID NO: 80 - DNA, 241 bp, Artificial Sequence
  DOK7 (-17,061), HGFAC (+4,363)
gcacaagaagaggacgttcctgcggccacgtatcatcggcggctcctcctcgctgcccggctcgcacccctggctggccgccatctacatcggggacagcttctgcgccgggagcctggtccacacctgctgggtggtgtcggccgcccactgcttctcccacaggtgcacctcctctgggccccagtcacctgccctgaggccccacacaccatccagcgtcactatgcgcctgtcccca

SEQ ID NO: 81 - DNA, 306 bp, Artificial Sequence
  EVC (-2,765), EVC2 (+135)
ccttacctgcgtgctgctctcgggccccgccccgctccgccccggagggatcctcaggccgggcccagacctaggagccacctggggatcccggggtggctgcgcgccgagggggcgccagcggggacgtgagctggcgccgagacagcctcggccccccagcgccagggccactgccaggagacccccggccagcacccacgtggggcgcccccgggagcccgaggggtccatcgcctgtcgggacccgctacctcaaagcggcgggtgccgccgagtcgctggagcttccggaccccaggcccg

SEQ ID NO: 82 - DNA, 200 bp, Artificial Sequence
  HMX1 (+13,601), CPZ (+265,555)
ccaagccggtcgaggcccccgtccatttgggggaaatggattttcgcgatttaagaaacaaacccaaatcaaatgagcgaggcccggatgtgctgacgctgcggttacgcgcgcggagctggagccccgagagcgctctaggaaaggcgcagcggcgaccgcgggagggggtgagaagccgaggcagagaggtccggaga

SEQ ID NO: 83 - DNA, 282 bp, Artificial Sequence
  IRX1 (+533)
cgcccgggagggagagactacgggtggacctggtccggaagaggaactagaaaggtccgggggcaggttcccggtggccgaggccgcggcccccggggacgcaagagggctgggaggccgggcgggtgacggctgggccatctcggcctgggaaagcggaaggcccgggccagggagcgggtagcgagtgaattcagagaggccgcagaagcaggcccgtggagcggtgcccgcgctggaggtcgggggcaaactcgcctggctcggccagggcgcccgggc

SEQ ID NO: 84 - DNA, 214 bp, Artificial Sequence
  IRX1 (+3,659)
acgaggagatcgacctggaaagcatcgacattgacaagatcgacgagcacgatggcgaccagagcaacgaggatgacgaggacaaggccgaggctccgcacgcgcccgcagccccttctgctcttgcccgggaccaaggctcgccgctggcagcagccgacgttctcaagccccaggactcgcccttgggcctggcaaaggaggccccagagcc

SEQ ID NO: 85 - DNA, 200 bp, Artificial Sequence
  GDNF (-4,347)
ccggggtgggggaggggaggcgcggggccccgggagggaggggtcgggaggcgtcggctgggcctggcggtgggggaggagaggagagcagcgaggaggccctggagttcccgaggcggggggccggggtgcgagtgggcgacgcgaggcgcccctccctgggctgcagggagagcgctgagagcgcggagacgccgcgg

SEQ ID NO: 86 - DNA, 200 bp, Artificial Sequence
  AGGF1 (-76,519), CRHBP (+1,153)
gctcgcggacatctcggggaaggggctggccggaaccgccaggggcgcggtccccttagctaaggatcggtccgcggaggcgcgccaggagcgggagagggtggcgcgcccggggcgcaggaacccagcgcagcctaggctggaagtcggggcgctgggcactacagagcccgggaatggggcgcgcggagagcggccgc

SEQ ID NO: 87 - DNA, 200 bp, Artificial Sequence
  PITX1 (+5,529), CATSPER3 (+60,863)
cggcgcggtgagctggggcttgcgagccggggccccgcgtgcgtcctccgcgcccgcgcccgcgcccttccccgctccggccgccggcccgcgtggtgcggcggggcggtcagctgttgtactggcacgcgttgaggcccgaggccgggccctgcaggccgccgtagccaaacgacgagtgctgtttggacttgagccgc

SEQ ID NO: 88 - DNA, 377 bp, Artificial Sequence
  NEUROG1 (+837)
atctattgcctgctgactaggggagggggaaagtaacagtgtctacaaagggcctagtggtaaggaatgaaacagggcgttgtgtggagcaagtctttgggcaggcttgggaaggagaaaacagggtcgccggggcggtaggtgaagtcttcggaggcggctgggctactggggtcagagagcggggaggcggcggcggcacctgagccccaggactccgcgtcgctggcggggcttgggggaccgggcaggcaggggacgcactgcggcggcaggaggcgctcccgggcaccgcctccgggcagcccttgatccgccaggcgcagtgtctcggccagagcccagatgtagttgtaggcgaagcgcagcgtctcgat

SEQ ID NO: 89 - DNA, 203 bp, Artificial Sequence
  NPM1 (-72,025), TLX3 (+6,339)
aggcgtctgcaaggaggggcgagtctgcccggtccgggcagggagtgaggccacagtcagttctccctaggaggccgcgcagcgggtagggtatgggactgggggacgcaacggggacctggccgaatcagagccctcagcagagaacgccgaaaactctggggccggccgctcgcttcccgctagtgggaatggtttccggt

SEQ ID NO: 90 - DNA, 364 bp, Artificial Sequence
  NKX2-5 (+2,624), BNIP1 (+88,291)
ccacgcgggtcccttccctaccaggctcggataccatgcagcgtggacactcccgagttgctctgcggaatcccggggctctgaaccgcattcaagtccccgacgccgaagttcacgaagttgttgttggcggcggcagtggccggctgcgctggggaaggcccggcggggtaagcggcagtgcagctgtagccagggctgcaggccgcgccgccgtaacccggataggcggggtaggcgttataaccgtagggattgaggcccacgccgtaggcaggcgcgtagggcgccgagtcccctaggcatggcttgccatcgcgcaccagcactggcaccgcgatcctgcgggcaggcggcggcggcg

SEQ ID NO: 91 - DNA, 396 bp, Artificial Sequence
  PROP1 (+11,614), B4GALT7 (+384,528)
agagctcgtcccacgacggagcaggtccctttgcatcccgcggggccgccaggtgcaattttcgctgggccgacggcgcggagatgggccagagtccggccatccagaagtgcctggagcgcacagcaaggccctgccctcggctccgtgaaggtgagggggtaaagtcggcccggagtccccgggggtgcaggaggggccccgcgggttccagcagaccctcgacggaacgttccaggcaggcgagatctcgcacagaatctgcccttttaaaggctcggctttgtcctcgttaaacttgcgtctggcaacgcgaccgctgcggctcccgagcaagattagagggtttccgctcgcaggggcgcgcccggggaccgcgcctccccgcctggtctc

SEQ ID NO: 92 - DNA, 200 bp, Artificial Sequence
  IRF4 (-200)
tcgcacctcgcccttcgcgggaaacggccccagtgacagtccccgaagcggcgcgcgcccggctggaggtgcgctctccgggcgcggcgcgcggagggtcgccaagggcgcgggaaccccaccccggccgcggcagcccccagccttcacgccggccctgaggctcgcccgcccggccggccccggctctcggcttgcaa

SEQ ID NO: 93 - DNA, 200 bp, Artificial Sequence
  FOXF2 (-11,028), FOXQ1 (+66,366)
tggcgcggccggggcctggagaagcagcgctgagtccgacaccgcccaccaggcccctcttggagaactagacaggcgacagcactcaggaccccggctgcggccggcgccgcggcagccacgcgctccagcccgcgtgcacctgcttcgctccgccgcgctcccggcttaagccggcggctccggggtcctgccccgac

SEQ ID NO: 94 - DNA, 200 bp, Artificial Sequence
  FOXC1 (+14,713), GMDS (+620,532)
tggggcgcgaggccccaggactcggggacccctctacctcggcggcagcgtgcgaccctctttctaacgcggccgtggatgtttcttcccgggccgcagccaagcgcggttcttcctgggcggtggctttgggcttttcgtacccacagtcaagtcagttcacgtcgcctcccgcacacacgcgttcataaaacgaaact

SEQ ID NO: 95 - DNA, 200 bp, Artificial Sequence
  MOCS1 (-413,413), LRFN2 (+246,336)
tggtggtggggcggatactccagcatccccctttttgggcagaaagtttcctgcttgcttgtcttgcttcccttgccagccagggaatgggtcaggggcagggtctctatccagcctgcatcctggcaaggagccaacattccataaatctatgtttgataaattagtgaaagagacgataccatgcaaagataacacac

SEQ ID NO: 96 - DNA, 200 bp, Artificial Sequence
  POU3F2 (+9,136), FBXL4 (+104,086)
tgggaaggcgaccaagggcagcagcaggggctcctgcggggcgcaggtctgtgctggcgccgggcctggcctctgcaggctcggcggagcctcccgattgctcccgccgcacccgcccgcggccactcacccggccccgcggccagcccgggcggggtcgcacgcaaacaaggatgcttctatttactcgcctctgcctg

SEQ ID NO: 97 - DNA, 239 bp, Artificial Sequence
  CCR6 (+8,741), GPR31 (+26,819)
ccgtccctccctttttggcccccgctgctcttcccatcgtcatcaactcagcctccacgtgatggggaggtcactccctcccatccggtcccagccccactcacctgggaacccgtgccgctggccccaccttggcctagcatccgtccaaccctgcagcgaccgctccccacagcccctgctcccttgttctccagagccgcgcccctgctgcaggcctccccctcgctgtccccaag

SEQ ID NO: 98 - DNA, 200 bp, Artificial Sequence
  TBX20 (-3,712)
cagcgcgcggctccgtgccccgtggggagcgcgcggcgcggccttggatttcaccgcgagtcgggagggcgggtctgagccttgcctcccaggatccttccgacgaacaccccgcgggttttagtttatcgagccaaagtggtcccggagaagcgctccctcgcagccaagctgcaagaagtggccgggaacctacaggc

SEQ ID NO: 99 - DNA, 316 bp, Artificial Sequence
  TBX20 (-7,495), HERPUD2 (+433,492)
gctgctcggagccttagtttccctagttgtgaagagggagggtgtgaccatggcccggagctctccgaaaggctgtgcggattgctcggtggcgggatgtggagcgcgtcttctatgatgccaggtgctggccaagcgctcgatgcaggctgctccagttaggtcgatgcgatggcgggaagcactttcctctgcaatggagagacgccgacaccccgagcccgaaggcttgcaaggcgcgctctcgccactggggtcggggatccgtgggttctctatcccgcttacccactccatccttagcagctgtcgtcgg

SEQ ID NO: 100 - DNA, 200 bp, Artificial Sequence
  VIPR2 (+544)
ggaccgagaggcatctgcggccaacgccaaccccgatctccccgtgaaacgcgcagcccgcgcaggcgcccgcagctcccagctcccgggacggccccgaacgagctcatcgttgacgcgtccaggaagaaacgatcccgtttccagcaaaccccggacggtggggcgcggggaagggcgcaggcagcctcccaacccga

SEQ ID NO: 101 - DNA, 200 bp, Artificial Sequence
  LZTS1 (-214,206)
cacttgcggagagctcggaacactccgccgagaatgacttttggagccatttggcagagattagggaaaagaataagtggacacgctccagttatgaagaaaagacatatggggatttagattatgaacagacggaagaggaagaatgaggaatcattctttggagataaagactctccggaacagaagcgatgctgaaa

SEQ ID NO: 102 - DNA, 283 bp, Artificial Sequence
  NKX2-6 (-54)
gcgaagccgcggggcagctccgctcgcgctccagtcgcaggatgtccttgaccgagaagggggtggaggtgacggggctcagcagcatcccgaaggcggatggggcggggccgaggaggtccgggtgaggagcggcaccctgaacttcccgtcttgtcgctgcaggccccgcagacagacccaagctctgggacagacgcccagcgtcccagacagcgccttcctctgggccatgctggtaggcccgggtccagggccgggtgacgagaccgtagccccccat

SEQ ID NO: 103 - DNA, 200 bp, Artificial Sequence
  NKX2-6 (-40)
ctccagtcgcaggatgtccttgaccgagaagggggtggaggtgacggggctcagcagcatcccgaaggcggatggggcggggccgaggaggtccgggtgaggagcggcaccctgaacttcccgtcttgtcgctgcaggccccgcagacagacccaagctctgggacagacgcccagcgtcccagacagcgccttcctctg

SEQ ID NO: 104 - DNA, 238 bp, Artificial Sequence
  PENK (+36)
gcattcggcccgcacggtcgccaggagcccggggccgagcaacagcagccaagtgcaaagtgtcaggaaccgcgccatggactgcgaggagagagggacgcgtgcttcgagcctgcctgggcgcagaacggggtccctcggcaggaccctcgccgcgacagcctcagcaggggatcgtcgagcaaaagcccgcaggaatgctcctttctggggccccgccctcccggccgacagcttt

SEQ ID NO: 105 - DNA, 265 bp, Artificial Sequence
  PRDM14 (-99)
ccgcggggcatcgacaggtcgagggtagggaattgacccggcccacgcagatccccgcgtcgtcttctccccgcccaccgcagccattggccgactctcgactcgccctctgtcccctggggtcgctcacttaactcatcagttttccaaaccctccctgggaccctagtggcgagcactcgccgctggccttctagggcaggcagtattgccgctccaggcgtgcggagtcggggagaaaaaaaccgaacacgtgtgctaccca

SEQ ID NO: 106 - DNA, 200 bp, Artificial Sequence
  VPS13B (-38,563), OSR2 (+30,261)
gggagtccgcccttccctgcgccttcgggaccggcaggaggcgctgcgcgggcgaattaaaagaaaaggaaaagctcgtagtggaggtgttaccgcatcctgcctttggacgctactcttagttgagtgacccgattcggaccttaggggcgttagggtctcctccaccgcctccctcccctgttaaaagtgtgtgtgtg

SEQ ID NO: 107 - DNA, 450 bp, Artificial Sequence
  NEK6 (-241,823), LHX2 (+4,530)
gaggcagggcggcgagggtcccaagagaaagggctggctgtggcccggggcgccgagctcggcctggagtgcggcctgacctcgtgaaatgtcccaagggcggcaggcttggggaactcgggcttggggaactcaggaaagcaaaggctgcggttccttttgctcggcccgatcctcctttaaagacaggtctcagttttcccggactttttcctccgagtttcctggcgcctgctggggtgagggccgtgaccctcggaagcgagccccccgggcggggacgagaccggagcaggcctggcctcgcgccggggtggggtggggtggggtgaggtggggggcttggttcggatttccggcatctttgaaccccaggccattcccggagaagctctgccccctcccgcgcccctccctgctcaggacagctgcagaggttctgagttccgg

SEQ ID NO: 108 - DNA, 363 bp, Artificial Sequence
  DDIT4 (+35,651), DNAJB12 (+45,578)
tgattacagtccggagccatgatgggctcccagttgccaccttttccaagaagctgacttttgaggaatccgcctggccacgggaatcacaccatgtttgcactgccctcagctgttgattacaccctcatccgcgcaaccggcatccaggaagaacactttcttcctcacagggtgtctcctctcctgttttcatgtttatggcatcaggtggtttgcagagtgctccacacccagacatgtgcgtccagtgaggtcagctgagaaaacaacagcttgcccaccaccctgctcccccctcattctgggagctacaggctggggccacggtcacccctgggcacacgcccccacccccacctt

SEQ ID NO: 109 - DNA, 327 bp, Artificial Sequence
  CRTAC1 (-215)
cggcgagggcgggcgccccccgcgccccgccactgcgtcgcgtaaccttcaggcggcagcgaggcctggcgaggaggggagagggcgcctggctgggcgctgggggccccaggccggagggaagcgagggtccctcgggaggcagcgcagggaaggaacgcgaagggggaggggagggcggcgagccccaggaccccgcggccacccctgcgcgcaggaccgagggtggaggcgggagcggctgcactgccttcccatttccccccaggatagcgatctggcgtcgccgggccgggccaaagcggccgagcgagccgcgctgatggc

SEQ ID NO: 110 - DNA, 200 bp, Artificial Sequence
  PAX2 (-8,064), HIF1AN (+201,788)
gagctgcggagctgggcaggagacagggctgtgtttgggaaaaggaaaccgcacttcgaggcggctccgcagagcagagctgcagagtcttccgccctcccagccgccttctccctttgcctctttctcttttcaccgccccctccctcatctcttcggtagccacgtttggccggggcacaactccctggaggccctgc

SEQ ID NO: 111 - DNA, 200 bp, Artificial Sequence
  ELOVL3 (+478)
ggtggcattgaatgcccacaatgattttcttacagagcagagttatgggactcccttgtactggcttcacactacctttgtccgaggtgcaggtagtatgtggcacctcaaagagattagagctgaaagcaagcaagcagaaataagaggatgagggagaacgtggaaatatacagaagtcaaagagagcgtgtagtgag

SEQ ID NO: 112 - DNA, 204 bp, Artificial Sequence
  INA (-228)
cgacagagctgtgtggtttccggatgggaaacctcagtcgtttaggcacccctccgctcgagtcacttccgaagcagtcgattcttggggagaagcgctgcggaaaggggcgactccgatgcagatggccctgtcccggcgccccaggtcgtcgcgcgcgcagctgcggtagtcactgcgcctccccgcccccactcctggatg

SEQ ID NO: 113 - DNA, 280 bp, Artificial Sequence
  HMX2 (-10,758), HMX3 (+1,402)
gaagcggcgccaggcgcggccggggcgagcgtaggggcggcggcggccactccgggcgcagaagactggaagaagggcgctgaaagtccagagaagaagccggcgtgccgcaagaagaagacgcgcacagtcttctcgcgcagccaggtcttccagctcgagtccaccttcgacatgaagcgctatctgagcagctcggagcgagccggcctggccgcgtccctgcacctcaccgagacgcaggtcaagatctggttccagaaccgccgcaacaagtgga

SEQ ID NO: 114 - DNA, 200 bp, Artificial Sequence
  HMX2 (-2,034)
atatttacagttcaggaaggttcgaccaactttccctgcctgcccccagctttcttccccagcggggtggctggcactgctccccgagttagctggccagttcccctcggggctgccttgaccctggctccggaggcagcgcctagctcaggatgtctgcgagaagcggatggttagtgagaatccgacgattctttcgc

SEQ ID NO: 115 - DNA, 200 bp, Artificial Sequence
  MKI67 (-160,359)
cgtagttgtctcctggctcctggggtccgcggagctctagatgtacctgcagctcctcccgagtcctgcaagccacccttgtccctcttctcccgctcaccccccggcccccccatctcttttgctattccggggaaggccacgcagggtgcaacccggacgcgcccccgggggaagcccgcgacgcagcagccacaccc

SEQ ID NO: 116 - DNA, 214 bp, Artificial Sequence
  DPYSL4 (+15,897), STK32C (+105,143)
cctgccgtggtcataagtcagggccgagtggcgctggaggacgggaagatgtttgtcaccccgggggcgggccgcttcgtccctcggaaaacattcccggactttgtctacaagaggatcaaagctcgcaacagggtagggcggcacccgcaagggtgttgtgcaggtaggcaggtgggcgctgagttctaggcccagaacgcacccctggtca

SEQ ID NO: 117 - DNA, 314 bp, Artificial Sequence
  INS (+296), INS-IGF2 (+301)
gcggccaggggcagcaatgggcagttggctcaccctgcaggtcctctgcctcccggcgggtcttgggtgtgtagaagaagcctcgttccccgcacactaggtagagagcttccaccaggtgtgagccgcacaggtgttggttcacaaaggctgcggctgggtcaggtccccagagggccagcagcgccagcaggggcaggaggcgcatccacagggccatggcagaaggacagtgatctgggagacaggcagggctgaggcaggctgaaggccaggtgccctgccttggggcccctgggctcacccccacatgc

SEQ ID NO: 118 - DNA, 319 bp, Artificial Sequence
  ASCL2 (-310)
ccagggtctcagccaatcgtgggccacccgtttggccaatcgcgcagggcgcggctccacgcccggccccattgaggaagcgcgtacgcgtggcgcgtggctcacggggagcatcgctaacaaagctgggttcctgctgggccccgccctgctcctcgcccccgcgactgggctgggcgcgctgtcccctagcgcagctatgtcccgagcgcgcccccacctgtgcgttaatctactgggaatgggggtggactgcgccttacctggggcggggtggggcttaaggagtggtcgagactgaggcggggtgggaggttca

SEQ ID NO: 119 - DNA, 330 bp, Artificial Sequence
  PAX6 (-52)
ccggttcccacacttctcaccgccgctcggcaggggaagtggcagatctgacagccgcgttctacgcgaggacctgccccagagtttaaatgtcaatgataagaaaagagggtgctcaggcaggcgctaactttccttaatatccacgccagcgccgtcctcattggctgcccggcccgcgtgacgtcatggcggctagagttgggcacagctctgcgccgactagttttccggccgggcgggagcctgcttctccccacccagggtccggccggctccaacccctgctttggccttccttggcccggcctgtgactgctctagcccggc

SEQ ID NO: 120 - DNA, 200 bp, Artificial Sequence
  RELT (+12,570), FAM168A (+209,349)
tgggtgttggttgcaaccctgtcatcacggacacaggccgccacacgcgcttccttcccctgctgatgcctcggggcacctggcagtttaaggaaggggaaggaagcccttcctcctctgggaagcctcccagcctgcagagccttcttcctgccttcctgcctgtgctgccccgtgaggccggctcccaggcagggcag

SEQ ID NO: 121 - DNA, 200 bp, Artificial Sequence
  OPCML (-258)
acgagacgcggggacgcgcggacgccacgctcagcggccgcccccggcctccgcgccgccttcctcccgggagcagccccgacgcgcgcgggcccggaccgccggggttgtcatggcagcagctccatccctgaccgccactttctcccggtgccgcctcggagcgagcgggctggcgggcggcgcggactgcgcgctca

SEQ ID NO: 122 - DNA, 344 bp, Artificial Sequence
  ACVR1B (-33,666), ACVRL1 (+10,617)
ccatcagccccacacggactcgcggcgcattataaacactgtaatctggtgtcagccccggcactgattaaaggcccattagacacattcaggcctctgtgcagcactgattagggcgtgagcggcacaggggccggcctggaagctggccatggggagaacagctggcgaaggctctatcgaggttgcggcctgtgtggccatggcccccagcctcaggctgggaaacaggatggggcacggggctgtctgcggctccaccggcattgttttcagaaagctcctactaaaaactgtgaacttgggataccaagaggagggggtcagtgctggctgcaggagtc

SEQ ID NO: 123 - DNA, 311 bp, Artificial Sequence
  AVPR1A (+529)
ctcgatcatggagaagacgaagtactgcggcgtgctcagcacgaagctcagcacccaggcggccgcgatcatgaggcgcgagcggcgcgcgggctgttgcagagtcttgagcgggtggcacaccgcgatgtagcggtcggctgtcatgactaccagcatgtaggccgacgcaaacatgccgaacacctgcaggtgcttcaccacgcggcacagccagtcggggccgcggaagcggtaggtgatgtcccagcacatttgcggcagcacctggaagaatgccacggccaggtcggccaggctgaggtgtcgga

SEQ ID NO: 124 - DNA, 200 bp, Artificial Sequence
  LHX5 (+7,670), SDSL (+42,165)
accgggcagggacaaaccagcggacagagcagagcgcgaaatggttgagaccgggaagcgacctggccgggggaaactggatccgggccgcggcaggagcgactggtgggttgggccgggcggggcggccttggcgccctaaactcggtccctgcgccctaccaacccagtccaagtccttcgcctcgccaagtacggcc

SEQ ID NO: 125 - DNA, 200 bp, Artificial Sequence
  RAB20 (+27,350), COL4A2 (+227,116)
tgtttctctggggaagcctggctgccttattcacgtggactgctcacttgcttccctgggatggaggctgtctgcaaagctgaggctctccagagaggcctgtacagctcccccattttcaggctgtcccctgaggccgagcccctacaaagaggtgctgccaccgtgatgtacgagtgtgccggtcaagggtgccgacc

SEQ ID NO: 126 - DNA, 295 bp, Artificial Sequence
  CARKD (+9,535), CARS2 (+80,961)
cctggctgggtgtaatccgagctagtacgtttctcatgcacgtcaccagggctgagtaatgagcgctggacgcctgtgtctggcgggtgggcagcgatgccggagcgatccctgagtcggcctcttgtgctccttcatcagggcgcagacttgtcccacgtgttctgtgccagtgcggccgcacctgtgattaaggcctacagcccggagctgatcgtccacccagttctgtgagtcgctctgcgccggcttctcgtaggttctctttccctcctgcatcatttggggttttggc

SEQ ID NO: 127 - DNA, 212 bp, Artificial Sequence
  SOX1 (-10,416), TEX29 (+738,482)
gctggccggtaaaggctctcgggagaggggcgcggtgtctccacggtgactttccgtgaaggaggatggggtgtctccgcagctttggggccccaggaaagaacaggtgggtagatgtggtggccacggctagcggactcgccgcggggcacatttgtcattttcttatctgtgcgttcactcctcccccatcctcggcttttgggattggc

SEQ ID NO: 128 - DNA, 213 bp, Artificial Sequence
  SPACA7 (-271,785), SOX1 (+36,935)
ggcgctgggctgtgcgtttgcacaaatctgtgttccggcgggccggtgtcaaccctagtggggacacgggagaaagagcacgccagtaggccacgcggcgcgtgggcagtgcgcaacttctgtcggcgtccaggctgtacggccacgtttcagccggtgcccccaggccatggacacccagctccagggtcgctctgcgccctttctccccag

SEQ ID NO: 129 - DNA, 235 bp, Artificial Sequence
  SPACA7 (-270,565), SOX1 (+38,155)
ggacccggagcagcctgggtggagcgcggcctcgggaggccctgggtgcatcgcggcggggcctgggggggcccaggcgccggaggagccgtcggtgccggaatgcagcgtgtttcacttgggagaaacgttgccctcggtcccttgcctccctcctgttgtctcggtttttctggcttcgtccttcgtcccacccacccgttcccacctcaggtccctcccccaggatcccctc

SEQ ID NO: 130 - DNA, 266 bp, Artificial Sequence
  SFTA3 (-3,697)
cgtggtgcgccaggtccggagactggcctgcgctgcctggctggtggcccgggtgtgcgccaaggccggcgccaccgctgcccacggagatggccgctgccgccgcctgcgcggcctgcgcctggtgctgcgcctgctgctgcgcgtggccttgtaggctggcggcgcccggcgcgggggcacccgcctggcacggtttgccgtctttcaccaggaccggcaccgccacgcgtcgcggcgactgctgctgagcctgttgctgctgc

SEQ ID NO: 131 - DNA, 287 bp, Artificial Sequence
  SIX6 (+1,140), SIX1 (+139,371)
cgagcggctgcagccaagaacaggtcggtacctagaggcctccgcgctttgagcgcaccggggaggaggcgggtggaggcacctctggcgcccttacccagtccctggcgactccaattcagcaggagttgggagcgcggtctgtcttgggttaagagccctgcgttctgggctcctggccgggagttcccttgccggctctgcttccccacccgctggctccccacgcctgcgggcagctgcagcagctggtcccggtcaccaaaccaaggcttcactgggacgga

SEQ ID NO: 132 - DNA, 200 bp, Artificial Sequence
  INF2 (-53,425), TMEM179 (-30,565)
cccgggaagcagaagacggctcctggcacatctcctgggtgcatctgtggattgctggggcccccagcagctctcccaatccccagaaacccctcctggatctgctgtatccacctggagcctcttggtgcacagcggcacacacaatacctccactctccaccccgaaggatgcccactgcagcggggtcctcatccac

SEQ ID NO: 133 - DNA, 200 bp, Artificial Sequence
  CRIP2 (-5,544), MTA1 (+47,596)
aagtgctgggcctgccagtgtggatgtgcctggagccccttcgccaggcggctttcactgacggtgctggccagggcagcagggccggtttggcgacctggaggtggatatgggtagtggctgcccagcccagccaaccctgtccccttggggcattctctcgaggctgctgggtgtcctggcaggcacgtcctgtgggg

SEQ ID NO: 134 - DNA, 200 bp, Artificial Sequence
  PIAS1 (-232,067), SKOR1 (+2,408)
gagttggaacgcaggagggaaaggggaccatacccggtagcccgagggaaaaacgaggcgagaggggagaaggcgaccccgcgctgctacccgcggaagatttatggcgcctcccgggttccaaggacaggctgcgttcgtcgctgctgccaccgccggtagtcgccgtggccgctgcgccccctgcccaggcggcccgt

SEQ ID NO: 135 - DNA, 298 bp, Artificial Sequence
  PIAS1 (-224,987), SKOR1 (+9,488)
cccgctcaagtccagcgggcgcaccaacctttgccactccgtcggctttccctcttggccgcggggtagggctgggcgtctttgggccgccgcagggcgccaccctaatcgcctgtcatttctcggccgtcgcaggtgttcgcgcccgagagggatgagcacgtgaagagcgcggcggtggcgctggggcccgcggcctcctacgtctgcacccccgaggcccacggtaacgcctgtcgcggccgctggccactgtaatgggggaaccgcagacagagggccggggtcaaggaaggcc

SEQ ID NO: 136 - DNA, 393 bp, Artificial Sequence
  PIAS1 (-224,397), SKOR1 (+10,078)
gtttggccgcggggtcccctttggctaggccggatcggggcggaggatgggggcacatggccgcgcgcttgggtaccccagaagcgccagggtagctgaggcccatcgcggggtggtgggggccgccctgcacttgcgcgccttaccaggttcctcacagaggaggggttgggggcagcggaaaatcgggcaggtcgaggcagccgaaccccggacgatgtccccccacccaccccgaaggtcgcagcctgggccgcgttctcagcaggagtcgggcggacagacccggcggccacgcgcgctcgcggtgccccagtatctgcgcgcgatgtaggtcgctcgtccctggtgggctcggctgctcgcctagctcttttccaaggggctggggcg

SEQ ID NO: 137 - DNA, 624 bp, Artificial Sequence
  ISL2 (+6,367), SCAPER (+562,244)
ttatgcgggcgagggcgcgccccgctcccggaaccagccttggcctggcgcctgccgagccccgagccccactctcgctcggcgccgcgggccctcccggcgcttccttccccagcggtccgcggccctgggtgaggctcgaagccccgcgcgctgcccctggccctgcagcacagcagtgaggccaaccccggccagagcgggcggccgtgacgggccgtgccccgcgctgtccccggagtggatgcgcgacgtgatcaatccgcggcatttattaattccacagtctagacagaggcgggggccgggcggcggctgcttatctgcgtttggcatcacctgcaagcgatacaccgaggggccgcaacgagcccccgctaggagcgcggctgccgggaaaataagtccacccagaaccagtctggcgtgtccttggtttattttctttccagaccgaagtggagggggtcgggggtggcccgggtgggagggagctgggaatggcccctggatatgccgtgcccaggtcacttggtgtgacatttcaaacccctgcgacttgttttcttgaaaactggctttagtgatcgcaggaaataaccgagagatactgaatctccagta

SEQ ID NO: 138 - DNA, 260 bp, Artificial Sequence
  POLG (-74,438), RHCG (+87,328)
gactcttgctaatgactgggtaggaccctcggggtcctgcgacggtgctggagggtgttcccggctccgatgtggggaggcctgcgcggggactaggttctcgagaggcgagcgggcgcgccagagaacccgagactgctgcggggccggatgcgggatccctgggctgcggttctacgcagaaacgccaatggccatgcctccccagctcctcccagccccagtcactaggccggcgcctggcccggagatcctcccag

SEQ ID NO: 139 - DNA, 202 bp, Artificial Sequence
  NR2F2 (-16,885)
cttttacttggaaaataatggaggtaaggattttcttgcaagttttaaattctatggttttctaaagaaccatcgttgttttaagtattcagtgctctctggagtcaagaaaaagaaaaaggagacttcctctaatgctgagtgtcctcaagacagtctccaagaagcgggagccatgccctctcacagtgcactgtgtcac

SEQ ID NO: 140 - DNA, 323 bp, Artificial Sequence
  RAB40C (-9,067), PIGQ (+10,272)
cgtccctgggcgcggggtcctgctgatgcccggtgtgctggcccctccctacagctgttcatcgggactctgctcttcaccatcctgctcttcctcctgcctaccacagccctgtactacctggtgttcaccctggtgagctgagcacccacaggctgggcctggctgcagtgctctgtgtggcttctgccagcgctgcctgggagcagtcagctgtggggcgggctgtctcctgctgcaggccacgtgggtggcctttcaggaccctctgggcagtgagtgctgcgctctggagtgggcgaggccctatcctggccagtaag

SEQ ID NO: 141 - DNA, 309 bp, Artificial Sequence
  CPNE2 (-100,480), NLRC5 (+2,629)
atccaataggaccggtgtccttataagagaggagatggacacatgaagacagagacatacggggatcagacaatcatggacggaggaggaagagagtgcggcgatgcatctaggagccacaggacacctagaatggccagcagccggtgggaaccaggagaggcaaggacggatcctctcctccagccttcagagggagcccggccctgaccacacctcgatctcagactctgacctccagaactgcgagagaagaaatctcagttgttttaatgtacgcagcttgtggcactttgtgacagcagatac

SEQ ID NO: 142 - DNA, 258 bp, Artificial Sequence
  PSKH1 (-7,067), NRN1L (+1,400)
ccccgtccgaataacttgcacactctgtgcggtgccccggtgcatgttcgggagcgcggcacaggctccgaaaccaaccaggagacgctgcgggctacagcgcctgcactccccatggcccctgcgcccccactgctggcggctgctctggctctggcctacctcctgaggcctctggcctagcttgttgggttgggtagcagcgcccgtacctccagccctgctctggcggtggttgtccaggctctgcagagcgca

SEQ ID NO: 143 - DNA, 200 bp, Artificial Sequence
  SRR (-114,854), HIC1 (+132,540)
cccaggaacggttacctcaggaagggcagtctgagctggagctgcatggtctctgcctttagctgcctactgataatgtaaagccatcgtaacaagaactcagatttaattaactcagtctctctagtgtataactaacaggagcacagtcatcagttaagattggaaaaatacacatttaaaaatgatcttctgtctac

SEQ ID NO: 144 - DNA, 200 bp, Artificial Sequence
  HOXB9 (-92,914), PRAC1 (+3,131)
ccgcagtcggcgggtcgcctggaaagacgcgccggtttcccgggtcggatggctctccaggccgctatttcctccgccaccgagtagggagacgccccatttgcgaagtttaagtttccaggtcctgggaaggcagctgggaaacccgcggggctcggcagccgccctggtagcagccagggatcggatagcgcggcggg

SEQ ID NO: 145 - DNA, 206 bp, Artificial Sequence
  SMIM5 (-24,663), MYO15B (+9,414)
cagggccaggtaccacacctggatgctcctgggctgcctcccggtgcttgttcccaggccatcgggacgccctggctgggagcatcaccgagtgcctgccgcctgaggttcctgcccggcccagcctgactctcccagcagacattgacctgttccctttctccagcttcgtcgccatcggctttcaggtgggcgcccaggcctaa

SEQ ID NO: 146 - DNA, 781 bp, Artificial Sequence
  TNRC6C (-631,378), SEPT9 (+92,267)
gggcgggggcgcagcgcgcggggaggggccggcgcccgccttcctcccccattcattcagctgagccagggggcctaggggctcctccggcggctagctctgcactgcaggagcgcgggcgcggcgccccagccagcgcgcagggcccgggccccgccgggggcgcttcctcgccgctgccctccgcgcgacccgctgcccaccagccatcatgtcggaccccgcggtcaacgcgcagctggatgggatcatttcggacttcgaaggtgggtgctgggctggctgctgcggccgcggacgtgctggagaggaccctgcgggtgggcctggcgcgggacgggggtgcgctgaggggagacgggagtgcgctgaggggagacgggacccctaatccaggcgccctcccgctgagagcgccgcgcgcccccggccccgtgcccgcgccgcctacgtgggggaccctgttaggggcacccgcgtagaccctgcgcgccctcacaggaccctgtgctcgttctgcgcactgccgcctgggtttccttccttttattgttgtttgtgtttgccaagcgacagcgacctcctcgagggctcgcgaggctgcctcggaactctccaggacgcacagtttcactctgggaaatccatcggtcccctccctttggctctccccggcggctctcgggccccgcttggacccggcaacgggatagggaggtcgttcctcacctccgactgagtggacagccgcgtcctgctcgggtggacagccctcccctcc

SEQ ID NO: 147 - DNA, 390 bp, Artificial Sequence
  TBCD (+35,311), ZNF750 (+53,203)
aagagtgaggcgtgctgtcctgccgtttagggcagagcacccaggcggtttggcagcagcacctcagaactattcagagatttgccctcagcaagagtgagcaattgtctgacgcagccggctgaaatccctgggaagggaatgaatgaaactgccgtgaagcaacgcctggcggggccgggcttctggcagctcctggggccagcacgtcccttccagagcgtctgaagccctgggcggctgctggagcatctcgagtctttccagagtcatgtgtgttgtttccttctgtctcttggaagggtccgtttggtctgatccaggttgcctcagcaggaggaagtcgtgctgggtgctgagcgggtgggaggtttcaccttgggcttggca

SEQ ID NO: 148 - DNA, 200 bp, Artificial Sequence
  KCTD1 (-1,536)
tttcgggccgcggtgcggagaactcaggtgggtgcccggcaagttacctaccaggggctgttcccccgcgaccctcgccataagcgcagggacccgggggccgcgctggctccgggctgcgctcctggcttggcaggggaccaggcccacgctgcagcctgggagcggagccgccccccaggtctccccacctctgcggg

SEQ ID NO: 149 - DNA, 200 bp, Artificial Sequence
  SALL3 (-1,004)
gggtggggaacaccggggccctgcggtcccctccctttcctgtatttaagaagccgccggcggcgcagaggcccaggcgggctggcgcgggggcgaggcggcccggtggcagcagcgggcggggcgggcgctccggagtcggtggggcccgcgggttggggggcggggagaggggggagtggaagggagggggaacgcag

SEQ ID NO: 150 - DNA, 200 bp, Artificial Sequence
  CTDP1 (-183,273), NFATC1 (+96,192)
agtggagggctctgcccatgtctgtcagacagccatgttcttgccagggcagccagggccgggccactcaagctgggtgcttggctctccctgagctcgagcacgggcacgttcaggtgatcttcctgatagcaaagtgcgtttctgcgcatggactcctgaggagcagcgaggagctgactcacacattctgccaagcc

SEQ ID NO: 151 - DNA, 221 bp, Artificial Sequence
  ZNF554 (-19,119), THOP1 (+15,295)
ctcgcaggtcgggcactgccaagcttggctgccagccacttgctcagccctcccgtgtctcgggcagcacatcctaccctcagcttctggcactcaggagagacgacgggctacaatctgccgtaaagcacgtttcccagcctgcccctcagtgggtgcactgatcacccgcaccattcccgcagccacccacgccatcccgcggccacccgcaccgtccc

SEQ ID NO: 152 - DNA, 200 bp, Artificial Sequence
  CACTIN (-61,317), PIP5K1C (+12,347)
ggggccgacgggatgggtcagggtgcacagagcacacgccagcccctgggggaagcccggcccgtgcgggctgcgggagatcctgatgggccccgagctgaggctcccgcagccagggtctgcgcgtggtccccacctccttgcgcgctccgtctccagcacagcagaggtggacgcccctcgcggctggctccccagcg

SEQ ID NO: 153 - DNA, 200 bp, Artificial Sequence
  KDM4B (-56,963), PLIN3 (-44,389)
gattaatttctctggcttgcatgccataggagaccttcattagccctcttcccgtaagagacgtgatgacttgagtcttaagaatctgagttaacccgccctgccccgggaggaggcgatctggagaacttggggagttgacggtgcaagccgcgtgtgtgcagagaagaggcagggccgggctcgacagaggagctccg

SEQ ID NO: 154 - DNA, 324 bp, Artificial Sequence
  EPS15L1 (+70,842), KLF2 (+76,353)
aacacacacgccaagaacagccagggagcaaagcgaggagttctggcttctcgtaactcatgaaggatgaatgctcatcgtttaaatttagacgataaagctgatgatgacgggcccgggggcggctatggaaaccacctcattacgagtccacgagaaaagagagtatgggaggaaagagggaggcggtgcacccagcgggggccagacacaagagacagatgagctcgccagcagtgccttcccagcagcccaggggacgcgtgtgcttccccataaatccttgggactgaggacttggctgctgagaaaagaaacacatca

SEQ ID NO: 155 - DNA, 296 bp, Artificial Sequence
  EPS8L1 (+6,011), PPP1R12C (+35,647)
tcccctaggacatcctgaaccacgtgttcgacgacgtagagagctttgtatcgaggctgcagaagtcggcggaggcggccagggtgctggagcaccgggaacgcggccgcaggagccggcgccgggcggctgggggtaaggggcaccctggcgtgggatctgaaccccctcccgatctcttccaaatgtccccgctctccccaggctctcccctcccgccacttgccagggctgacctcaccgccatcttaaccgggtgtccacctctctctgcctgcctggtgctggccccgcgt

SEQ ID NO: 156 - DNA, 200 bp, Artificial Sequence
  NKX2-4 (-114,169), NKX2-2 (+1,829)
tgacatggtttgccgtccctgaccaagacgggcacggccacccggcgcggcgagggcaggggcgtcacctccatacctttctcggcccgggcgcgcttcatcttgtagcggtggttctggaaccagatcttgacctgcgtgggcgtgaggcggatgaggctggccaggtgttcgcgctcgggcgccgacaggtaccgctg

SEQ ID NO: 157 - DNA, 578 bp, Artificial Sequence
  TFAP2C (-1,962)
gatttgttctagctgccttccgtacagagggcgcggaggttgcgctccagttcgaacgcttacccattggaaagagggcagcgccggggtccagggaagctccttgggaatgaatggcctttgccaagcggttccggatcctctgggtcctttgggcccacggcacggtgctgcgcgagccctcagtgcccatcggctcccttcgcctcctgcgtagacgctcccaggcggggaggcatatcggttcctccgggcagctttggctagtgttgctgtgggaaaggagagccagggcctgggatgggggatgagcaccttcttgcccattccgggccccagcgtgcaggaggtaaacttgccagcacagacaagacagcttgttcaagctgcacctcaggccgggtcagagaataaaaccgagggctagaaggcccagaatgtcggacagcccagcggcacccgtcagggagtcccaggcgcccgaaagaggcgccgcacctctggcgagtctaggacccatcttcctggacctgtgctctggagtgcctgcgggcctgggtctaatttctgcttctggc

SEQ ID NO: 158 - DNA, 202 bp, Artificial Sequence
  RAE1 (-637)
tgggcgtgtgtgagtaataagaatcccttaacatttctacagacagttctattagtaagagtagttcacgtatgatttcacttgaccctaattaggaacagccctggcatcattttccccaccatgcagcaggaaactgaggcccaaagagccccgaggtgggctcagggtaccccagtgggcaaacagggagaggccaggg

SEQ ID NO: 159 - DNA, 249 bp, Artificial Sequence
  TNFRSF6B (+2,663), ARFRP1 (+8,326)
accaacctgcagaacacacacagggtcccctggagaggacgcggggacttccagggcccgactcctgtgagtcacagccccgcagctgctgcgccacccccaccctgactcatgccccttcccagcagctcctcccaggaccccatgtccttcccacatccgcaggaagggagtgcctggactctccaggcccacctggggagcccctcacctgcccaccagcccctgagcagcccagtaacaccatca

SEQ ID NO: 160 - DNA, 384 bp, Artificial Sequence
  MYH9 (-77,454), TXN2 (+16,560)
ggtcagtgtcctggaattggtcaaacaggatcaccaggaggattccgtgagcacagccagcatgactcacggccatgatcagcctcacgggcagaggctgccaacctgggatggccacagccaccggctcaccttgcagggcaacgcaccttttaaggagggagctggagcagcgcccgggtcctgcctctggccaaggcctctgccacacttctccacgcccacccgggcagagaggccagacccccactgggttcaaatttggcaccacttttcagacatgaccttgggcaagtcgatttctctgaactgtttttttcacttatgatatggaaataatacttgcctcacaagagtggaattcgatgaggtaatgtgtttaga

SEQ ID NO: 161 - DNA, 30 bp, Artificial Sequence
  ACTB probe
accaccacccaacacacaataacaaacaca

SEQ ID NO: 162 - DNA, 25 bp, Artificial Sequence
  ACTB Forward primer
tggaggaggtttagtaagttttttg

SEQ ID NO: 163 - DNA, 25 bp, Artificial Sequence
  ACTB Reverse primer
cctcccttaaaaattacaaaaacca

SEQ ID NO: 164 - DNA, 117 bp, Artificial Sequence
  TLX2 region 1
cgagcagggcctggtgagaagcgacgcggcgggcgccccgctgaccccgcgtctccctcccttaggcgccagacggcggaggagcgcgaggccgagcggcaccgcgcgggccggctg

SEQ ID NO: 165 - DNA, 21 bp, Artificial Sequence
  TLX2 probe1
cgggcgtttcgttgatttcgc

SEQ ID NO: 166 - DNA, 17 bp, Artificial Sequence
  TLX2 Forward primer 1
gtttggtgagaagcgac

SEQ ID NO: 167 - DNA, 17 bp, Artificial Sequence
  TLX2 Reverse primer 1
gccgtctaacgcctaaa

SEQ ID NO: 168 - DNA, 221 bp, Artificial Sequence
  TLX2 region 2
ccgcgtctccctcccttaaacgccaaacgacgaaaaaacgcgaaaccgaacgacaccgcgcgaaccgactactcctacatctacaacaaaacgcgttaccacgaccgctacgaccgccgctacccccgaaccctctctacctacacaactcgtcgctcttcgcgctacaaaacctacaaccctaaaccgaaaacaacaaaataacttcaatatccgaactc

SEQ ID NO: 169 - DNA, 17 bp, Artificial Sequence
  TLX2 probe2
cgaccgctacgaccgcc

SEQ ID NO: 170 - DNA, 18 bp, Artificial Sequence
  TLX2 Forward primer 2
catctacaacaaaacgcg

SEQ ID NO: 171 - DNA, 18 bp, Artificial Sequence
  TLX2 Reverse primer 2
gttttgtagcgcgaagag

SEQ ID NO: 172 - DNA, 102 bp, Artificial Sequence
  EBF2 region 1
gtacccacatgcacaagcgctcactcggccccgcacgcaagcagcgccccgcgcgcccggggccctcctcggataagggaggggtgacaaaagtctcccgct

SEQ ID NO: 173 - DNA, 18 bp, Artificial Sequence
  EBF2 probe1
agcgtttcgcgcgttcgg

SEQ ID NO: 174 - DNA, 20 bp, Artificial Sequence
  EBF2 Forward primer 1
cgtttattcggtttcgtacg

SEQ ID NO: 175 - DNA, 21 bp, Artificial Sequence
  EBF2 Reverse primer 1
cctcccttatccgaaaaaaac

SEQ ID NO: 176 - DNA, 196 bp, Artificial Sequence
  EBF2 region 2
gttcgttagtcggtaggggaaagttcgagggattttttagttttttttcggatcgcggcggaggtgtgagcgatgtgttgattatttatatttttatcgagcgtatattttgttgcggtcggcgtcgttatattttatacgtatattgacgtatttatatgtataagcgtttattcggtttcgtacgtaagtagcg

SEQ ID NO: 177 - DNA, 18 bp, Artificial Sequence
  EBF2 probe2
tttcggatcgcggcggag

SEQ ID NO: 178 - DNA, 18 bp, Artificial Sequence
  EBF2 Forward primer 2
gttcgttagtcggtaggg

SEQ ID NO: 179 - DNA, 20 bp, Artificial Sequence
  EBF2 Reverse primer 2
gcaacaaaatatacgctcga

SEQ ID NO: 180 - DNA, 148 bp, Artificial Sequence
  KCNA6 region 1
tgccgcgctccagagattgtgtcgtgggcgccgtcctagtggcggggagcgcacctccgagggggcatgagatcggagaaatcccttacgctggcggcgccgggggaggtccgtgggccggagggagagcaacaggatgcgggagact

SEQ ID NO: 181 - DNA, 21 bp, Artificial Sequence
  KCNA6 probe1
atcccttacgctaacgacgcc

SEQ ID NO: 182 - DNA, 18 bp, Artificial Sequence
  KCNA6 Forward primer 1
aacgcacctccgaaaaaa

SEQ ID NO: 183 - DNA, 21 bp, Artificial Sequence
  KCNA6 Reverse primer 1
tgtttttttttcggtttacgg

SEQ ID NO: 184 - DNA, 196 bp, Artificial Sequence
  KCNA6 region 2
aatccccaacgcccaaatcacctccccaaacccaaccttacaaaaaccaaaactttaaaactcacgaacccaacgaccaaatcaaaccgcgaaccgaaaaaaacgcgaaccccaccctaaaaaaaacgcaaccgaaaactaaaaaacgaataccgcgctccaaaaattatatcgtaaacgccgtcctaataacgaa

SEQ ID NO: 185 - DNA, 21 bp, Artificial Sequence
  KCNA6 probe2
ccgcgaaccgaaaaaaacgcg

SEQ ID NO: 186 - DNA, 21 bp, Artificial Sequence
  KCNA6 Forward primer 2
accaaaactttaaaactcacg

SEQ ID NO: 187 - DNA, 20 bp, Artificial Sequence
  KCNA6 Reverse primer 2
gatataatttttggagcgcg

SEQ ID NO: 188 - DNA, 203 bp, Artificial Sequence
  KCNA6 region 3
gacgccgaaaaaaatccgtaaaccgaaaaaaaaacaacaaaatacgaaaaacttcccgaaaaccgacgaaaacgaaaactactataataacgaacgactaataatcaatatctccgaactacgctttaaaacacaattacgcaccctatcgctatttccgaacacgctactcgaaaaccctaaccgacgaatccgcttcttcg

SEQ ID NO: 189 - DNA, 23 bp, Artificial Sequence
  KCNA6 probe3
ccgaacacgctactcgaaaaccc

SEQ ID NO: 190 - DNA, 19 bp, Artificial Sequence
  KCNA6 Forward primer 3
caatatctccgaactacgc

SEQ ID NO: 191 - DNA, 18 bp, Artificial Sequence
  KCNA6 Reverse primer 3
gaagaagcggattcgtcg

SEQ ID NO: 192 - DNA, 120 bp, Artificial Sequence
  CCNA1 region 1
cgttccttcctcttcctgggccacaatcttggctttcccgggccggcttcacgcagttgcgcaggagcccgcgggggaagacctctcgtggggacctcgagcacgacgtgcgaccctaaa

SEQ ID NO: 193 - DNA, 25 bp, Artificial Sequence
  CCNA1 probe1
cggttttacgtagttgcgtaggagt

SEQ ID NO: 194 - DNA, 24 bp, Artificial Sequence
  CCNA1 Forward primer 1
ggttataattttggttttttcggg

SEQ ID NO: 195 - DNA, 18 bp, Artificial Sequence
  CCNA1 Reverse primer 1
gaaaaatcttcccccgcg

SEQ ID NO: 196 - DNA, 196 bp, Artificial Sequence
  CCNA1 region 2
taggcgtttgagttttcgggtttttaggagtttttcgtataaggattttagggatttttttttttacgcggtcgggtcgttcgttcggtttttagttcggagagttgttatcgatttttttaacgttttaagttttagttttgtcgttcgcgtttttttttttttttgggttataattttggttttttcgggtcgg

SEQ ID NO: 197 - DNA, 20 bp, Artificial Sequence
  CCNA1 probe2
cgcggtcgggtcgttcgttc

SEQ ID NO: 198 - DNA, 18 bp, Artificial Sequence
  CCNA1 Forward primer 2
taggcgtttgagttttcg

SEQ ID NO: 199 - DNA, 19 bp, Artificial Sequence
  CCNA1 Reverse primer 2
gataacaactctccgaact

SEQ ID NO: 200 - DNA, 224 bp, Artificial Sequence
  CCNA1 region 3
cttcacgcaattacgcaaaaacccgcgaaaaaaaacctctcgtaaaaacctcgaacacgacgtacgaccctaaatccccacatctcctctaccgcctcgcaaaccacatacaccgaaaaccgaacgaaacaaacgcgacccgcaaaaacccccgcgataaaaacgcaacactaccgcgactacacttaaaacaaccccgccgcgtcccaaccgcctcccgacaa

SEQ ID NO: 201 - DNA, 18 bp, Artificial Sequence
  CCNA1 probe3
cgcgacccgcaaaaaccc

SEQ ID NO: 202 - DNA, 19 bp, Artificial Sequence
  CCNA1 Forward primer 3
cgtaaaaacctcgaacacg

SEQ ID NO: 203 - DNA, 18 bp, Artificial Sequence
  CCNA1 Reverse primer 3
tgttgcgtttttatcgcg

SEQ ID NO: 204 - DNA, 141 bp, Artificial Sequence
  FOXD3 region 1
tgggcgagggcgacgacgggctggaagagaaggacagcgacgcaggttgcgatagccccgcggggccgccggagctgcgcctggacgaggcggacgaggtgcccccggcggcaccccatcacggacagcctcagccgcccc

SEQ ID NO: 205 - DNA, 21 bp, Artificial Sequence
  FOXD3 probe1
cgcgaaaccgccgaaactacg

SEQ ID NO: 206 - DNA, 21 bp, Artificial Sequence
  FOXD3 Forward primer 1
gtatttcgttcgtttcgttta

SEQ ID NO: 207 - DNA, 19 bp, Artificial Sequence
  FOXD3 Reverse primer 1
acgcaaattacgataaccc

SEQ ID NO: 208 - DNA, 188 bp, Artificial Sequence
  TRIM58 region 1
ggtgcccggtgtgcctggatttcctgcaggagccggtcagcgtggactgcggccacagcttctgcctcaggtgcatctccgagttctgcgagaagtcggacggcgcgcagggcggcgtctacgcctgtccgcagtgccggggccccttccggccctcgggctttcgccccaaccggcagctggcgggc

SEQ ID NO: 209 - DNA, 19 bp, Artificial Sequence
  TRIM58 probe1
cgcgccgtccgacttctcg

SEQ ID NO: 210 - DNA, 21 bp, Artificial Sequence
  TRIM58 Forward primer 1
ggattgcggttatagtttttg

SEQ ID NO: 211 - DNA, 19 bp, Artificial Sequence
  TRIM58 Reverse primer 1
cgacactacgaacaaacgt

SEQ ID NO: 212 - DNA, 120 bp, Artificial Sequence
  HOXD10 region 1
caggacatggccaggcgctgccgcttgtccttcatgcgccggttctggaaccacacctgcggggagagacgcgccgcagcctgggttagggagcgccccgtgttcccagctcctgtccca

SEQ ID NO: 213 - DNA, 18 bp, Artificial Sequence
  HOXD10 probe1
acgcgtctctccccgcaa

SEQ ID NO: 214 - DNA, 18 bp, Artificial Sequence
  HOXD10 Forward primer 1
tccctaacccaaactacg

SEQ ID NO: 215 - DNA, 23 bp, Artificial Sequence
  HOXD10 Reverse primer 1
ttaggatatggttaggcgttgtc

SEQ ID NO: 216 - DNA, 154 bp, Artificial Sequence
  OLIG3 region 1
agtgaggcggcggacagcggtgacgaggcgttgccagatgagagcgcgccgcccaagatggggtgcaccgggtgcacggagttggccgcgtgcgcggggtggccggccgagtggcccacggtcccgcagtgaaaggccgagtggtggcccccat

SEQ ID NO: 217 - DNA, 21 bp, Artificial Sequence
  OLIG3 probe1
cacgaaattaaccgcgtacgc

SEQ ID NO: 218 - DNA, 20 bp, Artificial Sequence
  OLIG3 Forward primer 1
gcccaaaataaaatacaccg

SEQ ID NO: 219 - DNA, 20 bp, Artificial Sequence
  OLIG3 Reverse primer 1
gttattcggtcggttatttc

SEQ ID NO: 220 - DNA, 116 bp, Artificial Sequence
  EN2 region 1
cggcgcgatcagtagcgcccactaacagttcgttctgcacggcggagcgcgagaccgcggacccacggaagccccctcaatggtgtttgcgtcctcgccgccaccggcttggtagg

SEQ ID NO: 221 - DNA, 19 bp, Artificial Sequence
  EN2 probe1
aacgcgaaaccgcgaaccc

SEQ ID NO: 222 - DNA, 21 bp, Artificial Sequence
  EN2 Forward primer 1
cactaacaattcgttctacac

SEQ ID NO: 223 - DNA, 23 bp, Artificial Sequence
  EN2 Reverse primer 1
cgaggacgtaaatattattgagg

SEQ ID NO: 224 - DNA, 615 bp, Artificial Sequence
  CLEC11A region 1
cccatgagttcctggccccgcctccctccacccccggatgttttgtcctcgcccccttccagactctgaatgcatgaccccgcctccttctctacccggccccgcccacaggctgcctgaaggggctgcgcctgggccacaagtgcttcctgctctcgcgcgacttcgaagctcaggcggcggcgcaggcgcggtgcacggcgcggggcgggagcctggcgcagccggcagaccgccagcagatggaggcgctcactcggtacctgcgcgcggcgctcgctccctacaactggcccgtgtggctgggcgtgcacgatcggcgcgccgagggcctctacctcttcgaaaacggccagcgcgtgtccttcttcgcctggcatcgctcaccccgccccgagctcggcgcccagcccagcgcctcgccgcatccgctcagcccggaccagcccaacggtggcacgctcgagaactgcgtggcgcaggcctctgacgacggctcctggtgggaccacgactgccagcggcgtctctactacgtctgcgagttccccttctagcggggccggtaccccgcctccctgcccatcccaccacccggcctttccctgcgccgtg

SEQ ID NO: 225 - DNA, 23 bp, Artificial Sequence
  CLEC11A probe1
cgtcgtcaaaaacctacgccacg

SEQ ID NO: 226 - DNA, 19 bp, Artificial Sequence
  CLEC11A Forward primer 1
gtggtacgttcgagaattg

SEQ ID NO: 227 - DNA, 20 bp, Artificial Sequence
  CLEC11A Reverse primer 1
cgtaataaaaacgccgctaa

SEQ ID NO: 228 - DNA, 539 bp, Artificial Sequence
  TWIST1 region 1
gggctgcccggctcgtcgccgcctccgacgcccccacccgcggctccgccgggccccgcgccgccgcccgcgctgcgcctgctgctgcgccgcttgcgtcccccgcgcttgccgctcggcggctgctgccggtctggctcttcctcgctgttgctcaggctgtcgtcggccggcgagactggcgagctggacacgtcctgcatcatctctcgagcggcgacgcgtggcctcgcgggcccggggcagaggagaagagcggggcgcctcagcccgccagcttcccccgcgcgcggcgccggcccgggcgatgcggcccgcggaggagagagcaggaggacggacgggagggacctccgcggggagggcgcgcgggggaggcggggagggaggcgggagggggaggggacggtgtggatggccccgaggtccaaaaagaaagcgcccaacggctggacgcacaccccgccaggcctcctggaaacggtgccggtgctgcagagcccgcgaggtgtctgggagttgggcgagagctgcagact

SEQ ID NO: 229 - DNA, 19 bp, Artificial Sequence
  TWIST1 probe1
cgcgcttaccgctcgacga

SEQ ID NO: 230 - DNA, 19 bp, Artificial Sequence
  TWIST1 Forward primer 1
ctactactacgccgcttac

SEQ ID NO: 231 - DNA, 19 bp, Artificial Sequence
  TWIST1 Reverse primer 1
gcgaggaagagttagatcg

SEQ ID NO: 232 - DNA, 120 bp, Artificial Sequence
  EMX1 region 1
gacccggaaatccgttgggcactgaaggacttttcgaaccctgtagcgctgttgcttcgcggtccatcgtcgccgctgcagacggatgcgctccccggcggctctacgccctccagtccc

SEQ ID NO: 233 - DNA, 20 bp, Artificial Sequence
  EMX1 probe1
tcgtcgtcgttgtagacgga

SEQ ID NO: 234 - DNA, 18 bp, Artificial Sequence
  EMX1 Forward primer 1
gtagcgttgttgtttcgc

SEQ ID NO: 235 - DNA, 20 bp, Artificial Sequence
  EMX1 Reverse primer 1
gtaaaaccgccgaaaaacgc